European Patent Application EP 4 722 239 A2, published April 8, 2026. Title: COMPOSITIONS AND METHODS FOR ANTI-VIRUS CHIMERIC ANTIGEN RECEPTOR. Applicant: Christopher Rudd. Application EP 22858012.2, filed March 20, 2024. The sequence listing filed with the application follows.

SEQUENCE LISTING (117 sequences)

SEQ ID NO: 1 - protein, 229 aa, Synthetic construct
ESKYGPPCPSCPAPEFLGGPSVFLFPPKPKDTLMISRTPEVTCVVVDVSQEDPEVQFNWYVDGVEVHNAKTKPREEQFNSTYRVVSVLTVLHQDWLNGKEYKCKVSNKGLPSSIEKTISKAKGQPREPQVYTLPPSQEEMTKNQVSLTCLVKGFYPSDIAVEWESNGQPENNYKTTPPVLDSDGSFFLYSRLTVDKSRWQEGNVFSCSVMHEALHNHYTQKSLSLSLGK

SEQ ID NO: 2 - protein, 203 aa, Synthetic construct
NITNLCPFGEVFNATKFPSVYAWERKKISNCVADYSVLYNSTFFSTFKCYGVSATKLNDLCFSNVYADSFVVKGDDVRQIAPGQTGVIADYNYKLPDDFMGCVLAWNTRNIDATSTGNYNYKYRYLRHGKLRPFERDISNVPFSPDGKPCTPPALNCYWPLNDYGFYTTTGIGYQPYRVVVLSFELLNAPATVCGPKLSTDLI

SEQ ID NO: 3 - protein, 5 aa, Synthetic construct
TYWIG

SEQ ID NO: 4 - protein, 17 aa, Synthetic construct
IIYPGDSETRYSPSFQG

SEQ ID NO: 5 - protein, 10 aa, Synthetic construct
GSGISTPMDV

SEQ ID NO: 6 - protein, 17 aa, Synthetic construct
KSSQSVLYSSINKNYLA

SEQ ID NO: 7 - protein, 7 aa, Synthetic construct
WASTRES

SEQ ID NO: 8 - protein, 9 aa, Synthetic construct
QQYYSTPYT

SEQ ID NO: 9 - protein, 119 aa, Synthetic construct
EVQLVQSGTEVKKPGESLKISCKGSGYGFITYWIGWVRQMPGKGLEWMGIIYPGDSETRYSPSFQGQVTISADKSINTAYLQWSSLKASDTAIYYCAGGSGISTPMDVWGQGTTVTVSS

SEQ ID NO: 10 - protein, 113 aa, Synthetic construct
DIVMTQSPDSLAVSLGERATINCKSSQSVLYSSINKNYLAWYQQKPGQPPKLLIYWASTRESGVPDRFSGSGSGTDFTLTISSLQAEDVAVYYCQQYYSTPYTFGQGTKVEIK

SEQ ID NO: 11 - protein, 15 aa, Synthetic construct
GGGGSGGGGSGGGGS

SEQ ID NO: 12 - protein, 27 aa, Synthetic construct
FWVLVVVGGVLACYSLLVTVAFIIFWV

SEQ ID NO: 13 - protein, 41 aa, Synthetic construct
RSKRSRLLHSDYMNMTPRRPGPTRKHYQPYAPPRDFAAYRS

SEQ ID NO: 14 - protein, 112 aa, Synthetic construct
RVKFSRSADAPAYQQGQNQLYNELNLGRREEYDVLDKRRGRDPEMGGKPRRKNPQEGLYNELQKDKMAEAYSEIGMKGERRRGKGHDGLYQGLSTATKDTYDALHMQALPPR

SEQ ID NO: 15 - protein, 8 aa, Synthetic construct
DYKDDDDK

SEQ ID NO: 16 - protein, 6 aa, Synthetic construct
HHHHHH

SEQ ID NO: 17 - protein, 10 aa, Synthetic construct
EQKLISEEDL

SEQ ID NO: 18 - protein, 9 aa, Synthetic construct
YPYDVPDYA

SEQ ID NO: 19 - protein, 17 aa, Synthetic construct
MWLQSLLLLGTVACSIS

SEQ ID NO: 20 - protein, 684 aa, Synthetic construct
MALPVTALLLPLALLLHAARPDIVMTQSPDSLAVSLGERATINCKSSQSVLYSSINKNYLAWYQQKPGQPPKLLIYWASTRESGVPDRFSGSGSGTDFTLTISSLQAEDVAVYYCQQYYSTPYTFGQGTKVEIKGGGGSGGGGSGGGGSEVQLVQSGTEVKKPGESLKISCKGSGYGFITYWIGWVRQMPGKGLEWMGIIYPGDSETRYSPSFQGQVTISADKSINTAYLQWSSLKASDTAIYYCAGGSGISTPMDVWGQGTTVTVSSDYKDDDDKESKYGPPCPPCPAPPVAGPSVFLFPPKPKDTLMISRTPEVTCVVVDVSQEDPEVQFNWYVDGVEVHNAKTKPREEQFQSTYRVVSVLTVLHQDWLNGKEYKCKVSNKGLPSSIEKTISKAKGQPREPQVYTLPPSQEEMTKNQVSLTCLVKGFYPSDIAVEWESNGQPENNYKTTPPVLDSDGSFFLYSRLTVDKSRWQEGNVFSCSVMHEALHNHYTQKSLSLSLGKFWVLVVVGGVLACYSLLVTVAFIIFWVRSKRSRGGHSDYMNMTPRRPGPTRKHYQPYAPPRDFAAYRSRVKFSRSADAPAYQQGQNQLYNELNLGRREEYDVLDKRRGRDPEMGGKPRRKNPQEGLYNELQKDKMAEAYSEIGMKGERRRGKGHDGLYQGLSTATKDTYDALHMQALPPR

SEQ ID NO: 21 - DNA, 2055 bp, Synthetic construct
  source 1..2055: mol_type = other DNA
atggctctgcctgtgacagctctgctgctgcctctggctctgcttctgcatgccgccagacctgacatcgtgatgacacagagccctgacagcctggccgtgtctctgggagaaagagccaccatcaactgcaagagcagccagagcgtgctgtactccagcatcaacaagaactacctggcctggtatcagcagaagcccggccagcctcctaagctgctgatctactgggccagcaccagagaaagcggcgtgcccgatagattttctggcagcggctctggcaccgacttcaccctgacaattagctccctgcaggccgaggatgtggccgtgtactactgccagcagtactacagcaccccttacacctttggccagggcaccaaggtggaaatcaaaggcggcggaggatctggcggaggtggaagtggcggaggcggatctgaagttcagctggtgcagagcggcaccgaagtgaagaagcctggcgagagcctgaagatctcctgcaaaggctccggctacggcttcatcacctactggatcggctgggtccgacagatgcctggcaaaggccttgagtggatgggcatcatctaccccggcgacagcgagacaagatacagccctagcttccagggccaagtgaccatcagcgccgacaagagcatcaataccgcctacctgcagtggtccagcctgaaggcctctgacaccgccatctactattgtgccggcggaagcggcatcagcaccccaatggatgtttggggccagggaaccaccgtgaccgtttcttctgactacaaggacgacgacgacaaggaatctaagtacggccctccttgtcctccatgtcctgctccacctgtggccggaccctccgtgttcctgtttcctccaaagcctaaggacaccctgatgatcagcagaacccctgaagtgacctgcgtggtggtggacgtttcccaagaggaccctgaggtgcagttcaattggtacgtggacggcgtggaagtgcacaacgccaagaccaagcctagagaggaacagttccagagcacctacagagtggtgtccgtgctgaccgtgctgcaccaggattggctgaacggcaaagagtacaagtgcaaggtgtccaacaagggcctgcctagcagcatcgagaaaaccatcagcaaggccaagggccagccaagagaaccccaggtgtacacactgcctccaagccaagaggaaatgaccaagaaccaggtgtccctgacctgcctggtcaagggcttctacccttccgatatcgccgtggaatgggagagcaatggccagcctgagaacaactacaagaccacacctcctgtgctggacagcgacggctcattcttcctgtacagcagactgaccgtggacaagagcagatggcaagagggcaacgtgttcagctgcagcgtgatgcacgaggccctgcacaaccactacacccagaagtctctgagcctgagcctgggcaagttctgggtgctcgttgttgttggcggcgtgctggcctgttactctctgctggttaccgtggccttcatcatcttttgggtccgaagcaagcggagcagaggcggccacagcgactacatgaacatgacccctagacggcccggaccaaccagaaagcactaccagccttacgctcctcctagagacttcgccgcctaccggtccagagtgaagttcagcagatccgccgatgctcccgcctatcagcagggacagaaccagctgtacaacgagctgaacctggggagaagagaagagtacgacgtgctggacaagcggagaggcagagatcctgagatgggcggcaagcccagacggaagaatcctcaagagggcctgtataatgagctgcagaaagacaagatggccgaggcctacagcgagatcggaatgaagggcgagcgcagaagaggcaagggacacgatggactgtaccagggcctgagcaccgccaccaaggatacctatgatgccctgcacatgcaggccctgcctccaagataa

SEQ ID NO: 22 - protein, 120 aa, Synthetic construct
EVQLVESGGGLVQPGGSLRLSCAASGFTFSDHYMDWVRQAPGKGLEWVGRTRNKANSYTTEYAASVKGRFTISRDDSKNSLYLQMNSLKTEDTAVYYCARGISPFYFDYWGQGTLVTVSS

SEQ ID NO: 23 - protein, 228 aa, Synthetic construct
ESKYGPPCPPCPAPPVAGPSVFLFPPKPKDTLMISRTPEVTCVVVDVSQEDPEVQFNWYVDGVEVHNAKTKPREEQFQSTYRVVSVLTVLHQDWLNGKEYKCKVSNKGLPSSIEKTISKAKGQPREPQVYTLPPSQEEMTKNQVSLTCLVKGFYPSDIAVEWESNGQPENNYKTTPPVLDSDGSFFLYSRLTVDKSRWQEGNVFSCSVMHEALHNHYTQKSLSLSLGK

SEQ ID NO: 24 - protein, 41 aa, Synthetic construct
RSKRSRGGHSDYMNMTPRRPGPTRKHYQPYAPPRDFAAYRS

SEQ ID NO: 25 - protein, 21 aa, Synthetic construct
MALPVTALLLPLALLLHAARP

SEQ ID NO: 26 - protein, 25 aa, Synthetic construct
MNRGVPFRHLLLVLQLALLPAATQG

SEQ ID NO: 27 - protein, 18 aa, Synthetic construct
MLRLLLALNLFPSIQVTG

SEQ ID NO: 28 - protein, 222 aa, Synthetic construct
RVVPSGDVVRFPNITNLCPFGEVFNATKFPSVYAWERKKISNCVADYSVLYNSTFFSTFKCYGVSATKLNDLCFSNVYADSFVVKGDDVRQIAPGQTGVIADYNYKLPDDFMGCVLAWNTRNIDATSTGNYNYKYRYLRHGKLRPFERDISNVPFSPDGKPCTPPALNCYWPLNDYGFYTTTGIGYQPYRVVVLSFELLNAPATVCGPKLSTDLIKNQCVNF

SEQ ID NO: 29 - protein, 121 aa, Synthetic construct
QVQLVESGGGVVQPGRSLRLSCAASGFTFSSYIMHWVRQAPGKGLEWVAVISYDGSNEAYADSVKGRFTISRDNSKNTLYLQMSSLRAEDTGVYYCARETGDYSSSWYDSWGRGTLVTVSS

SEQ ID NO: 30 - protein, 111 aa, Synthetic construct
QLVLTQSPSASASLGASVKLTCTLSSGHSNYAIAWHQQQPEKGPRYLMKVNSDGSHTKGDGIPDRFSGSSSGAERYLTISSLQSEDEADYYCQTWGTGIQVFGGGTKLTVL

SEQ ID NO: 31 - protein, 119 aa, Synthetic construct
QVQLVESGGGVVQPGRSLRLSCAASGFTFSSYAMHWVRQAPGKGLEWVAVIPFDGRNKYYADSVTGRFTISRDNSKNTLYLQMNSLRAEDTAVYYCASSSGYLFHSDYWGQGTLVTVSS

SEQ ID NO: 32 - protein, 107 aa, Synthetic construct
DIQMTQSPSTLSASVGDRVTITCRASQSISNWLAWFQQKPGKAPKLLIYEASSLESGVPSRFSGSGSGTEFTLTISSLQPDDFATYYCQQYNSYPWTFGQGTKVEIK

SEQ ID NO: 33 - protein, 128 aa, Synthetic construct
EVQLVESGAEVKKPGASVKVSCKVSGYTLTELSMHWVRQAPGKGLEWMGGFDPEDGETMYAQKFQGRVTMTEDTSTDTAYMELSSLRSEDTAVYYCATSTAVAGTPDLFDYYYGMDVWGQGTTVTVSS

SEQ ID NO: 34 - protein, 112 aa, Synthetic construct
EIVMTQSPLSSPVTLGQPASISCRSSQSLVHSDGNTYLSWLQQRPGQPPRLLIYKISNRFSGVPDRFSGSGAGTDFTLKISRVEAEDVGVYYCTQATQFPYTFGQGTKVDIK

SEQ ID NO: 35 - protein, 505 aa, Synthetic construct
QLSLPSILPNENEKVVQLNSSFSLRCFGESEVSWQYPMSEEESSDVEIRNEENNSGLFVTVLEVSSASAAHTGLYTCYYNHTQTEENELEGRHIYIYVPDPDVAFVPLGMTDYLVIVEDDDSAIIPCRTTDPETPVTLHNSEGVVPASYDSRQGFNGTFTVGPYICEATVKGKKFQTIPFNVYALKATSELDLEMEALKTVYKSGETIVVTCAVFNNEVVDLQWTYPGEVKGKGITMLEEIKVPSIKLVYTLTVPEATVKDSGDYECAARQATREVKEMKKVTISVHEKGFIEIKPTFSQLEAVNLHEVKHFVVEVRAYPPPRISWLKNNLTLIENLTEITTDVEKIQEIRYRSKLKLIRAKEEDSGHYTIVAQNEDAVKSYTFELLTQVPSSILDLVDDHHGSTGGQTVRCTAEGTPLPDIEWMICKDIKKCNNETSWTILANNVSNIITEIHSRDRSTVEGRVTFAKVEETIAVRCLAKNLLGAENRELKLVAPTLRSELTVA

SEQ ID NO: 36 - protein, 500 aa, Synthetic construct
LVVTPPGPELVLNVSSTFVLTCSGSAPVVWERMSQEPPQEMAKAQDGTFSSVLTLTNLTGLDTGEYFCTHNDSRGLETDERKRLYIFVPDPTVGFLPNDAEELFIFLTEITEITIPCRVTDPQLVVTLHEKKGDVALPVPYDHQRGFSGIFEDRSYICKTTIGDREVDSDAYYVYRLQVSSINVSVNAVQTVVRQGENITLMCIVIGNEVVNFEWTYPRKESGRLVEPVTDFLLDMPYHIRSILHIPSAELEDSGTYTCNVTESVNDHQDEKAINITVVESGYVRLLGEVGTLQFAELHRSRTLQVVFEAYPPPTVLWFKDNRTLGDSSAGEIALSTRNVSETRYVSELTLVRVKVAEAGHYTMRAFHEDAEVQLSFQLQINVPVRVLELSESHPDSGEQTVRCRGRGMPQPNIIWSACRDLKRCPRELPPTLLGNSSEEESQLETNVTYWEEEQEFEVVSTLRLQHVDRPLSVRCTLRNAVGQDTQEVIVVPHSLPFKV

SEQ ID NO: 37 - protein, 144 aa, Synthetic construct
QEEDLPRPSISAEPGTVIPLGSHVTFVCRGPVGVQTFRLERESRSTYNDTEDVSQASPSESEARFRIDSVSEGNAGPYRCIYYKPPKWSEQSDYLELLVKETSGGPDSPDTEPGSSAGPTQRPSDNSHNEHAPASQGLKAEHLY

SEQ ID NO: 38 - protein, 107 aa, Synthetic construct
DIQMTQSPSSLSASVGDRVTITCRASQSISSYLNWYQQKPGKAPKLLIYAASSLQSGVPSRFSGSGSGTDFTLTISSLQPEDFATYYCQQSYSTPPTFGQGTKVEIK

SEQ ID NO: 39 - protein, 39 aa, Synthetic construct
IEVMYPPPYLDNEKSNGTIIHVKGKHLCPSPLFPGPSKP

SEQ ID NO: 40 - protein, 47 aa, Synthetic construct
KPTTTPAPRPPTPAPTIASQPLSLRPEACRPAAGGAVHTRGLDFACD

SEQ ID NO: 41 - protein, 119 aa, Synthetic construct
ESKYGPPCPPCPGQPREPQVYTLPPSQEEMTKNQVSLTCLVKGFYPSDIAVEWESNGQPENNYKTTPPVLDSDGSFFLYSRLTVDKSRWQEGNVFSCSVMHEALHNHYTQKSLSLSLGK

SEQ ID NO: 42 - protein, 48 aa, Synthetic construct
LLVKETSGGPDSPDTEPGSSAGPTQRPSDNSHNEHAPASQGLKAEHLY

SEQ ID NO: 43 - protein, 242 aa, Synthetic construct
DIQMTQSPSSLSASVGDRVTITCRASQSISSYLNWYQQKPGKAPKLLIYAASSLQSGVPSRFSGSGSGTDFTLTISSLQPEDFATYYCQQSYSTPPTFGQGTKVEIKGGGGSGGGGSGGGGSEVQLVESGGGLVQPGGSLRLSCAASGFTFSDHYMDWVRQAPGKGLEWVGRTRNKANSYTTEYAASVKGRFTISRDDSKNSLYLQMNSLKTEDTAVYYCARGISPFYFDYWGQGTLVTVSS

SEQ ID NO: 44 - protein, 7 aa, Synthetic construct
GFTFSSY

SEQ ID NO: 45 - protein, 6 aa, Synthetic construct
SYDGSN

SEQ ID NO: 46 - protein, 12 aa, Synthetic construct
ETGDYSSSWYDS

SEQ ID NO: 47 - protein, 12 aa, Synthetic construct
TLSSGHSNYAIA

SEQ ID NO: 48 - protein, 11 aa, Synthetic construct
VNSDGSHTKGD

SEQ ID NO: 49 - protein, 9 aa, Synthetic construct
QTWGTGIQV

SEQ ID NO: 50 - RNA, 2055 nt, Synthetic construct
  source 1..2055: mol_type = other RNA
atggctctgcctgtgacagctctgctgctgcctctggctctgcttctgcatgccgccagacctgacatcgtgatgacacagagccctgacagcctggccgtgtctctgggagaaagagccaccatcaactgcaagagcagccagagcgtgctgtactccagcatcaacaagaactacctggcctggtatcagcagaagcccggccagcctcctaagctgctgatctactgggccagcaccagagaaagcggcgtgcccgatagattttctggcagcggctctggcaccgacttcaccctgacaattagctccctgcaggccgaggatgtggccgtgtactactgccagcagtactacagcaccccttacacctttggccagggcaccaaggtggaaatcaaaggcggcggaggatctggcggaggtggaagtggcggaggcggatctgaagttcagctggtgcagagcggcaccgaagtgaagaagcctggcgagagcctgaagatctcctgcaaaggctccggctacggcttcatcacctactggatcggctgggtccgacagatgcctggcaaaggccttgagtggatgggcatcatctaccccggcgacagcgagacaagatacagccctagcttccagggccaagtgaccatcagcgccgacaagagcatcaataccgcctacctgcagtggtccagcctgaaggcctctgacaccgccatctactattgtgccggcggaagcggcatcagcaccccaatggatgtttggggccagggaaccaccgtgaccgtttcttctgactacaaggacgacgacgacaaggaatctaagtacggccctccttgtcctccatgtcctgctccacctgtggccggaccctccgtgttcctgtttcctccaaagcctaaggacaccctgatgatcagcagaacccctgaagtgacctgcgtggtggtggacgtttcccaagaggaccctgaggtgcagttcaattggtacgtggacggcgtggaagtgcacaacgccaagaccaagcctagagaggaacagttccagagcacctacagagtggtgtccgtgctgaccgtgctgcaccaggattggctgaacggcaaagagtacaagtgcaaggtgtccaacaagggcctgcctagcagcatcgagaaaaccatcagcaaggccaagggccagccaagagaaccccaggtgtacacactgcctccaagccaagaggaaatgaccaagaaccaggtgtccctgacctgcctggtcaagggcttctacccttccgatatcgccgtggaatgggagagcaatggccagcctgagaacaactacaagaccacacctcctgtgctggacagcgacggctcattcttcctgtacagcagactgaccgtggacaagagcagatggcaagagggcaacgtgttcagctgcagcgtgatgcacgaggccctgcacaaccactacacccagaagtctctgagcctgagcctgggcaagttctgggtgctcgttgttgttggcggcgtgctggcctgttactctctgctggttaccgtggccttcatcatcttttgggtccgaagcaagcggagcagaggcggccacagcgactacatgaacatgacccctagacggcccggaccaaccagaaagcactaccagccttacgctcctcctagagacttcgccgcctaccggtccagagtgaagttcagcagatccgccgatgctcccgcctatcagcagggacagaaccagctgtacaacgagctgaacctggggagaagagaagagtacgacgtgctggacaagcggagaggcagagatcctgagatgggcggcaagcccagacggaagaatcctcaagagggcctgtataatgagctgcagaaagacaagatggccgaggcctacagcgagatcggaatgaagggcgagcgcagaagaggcaagggacacgatggactgtaccagggcctgagcaccgccaccaaggatacctatgatgccctgcacatgcaggccctgcctccaagataa

SEQ ID NO: 51 - DNA, 747 bp, Synthetic construct
  source 1..747: mol_type = other DNA
atggctctgcctgtgacagctctgctgctgcctctggctctgcttctgcatgccgccagacctgactacaaggacgacgacgacaagatcgaagtgatgtaccctcctccttacctggacaacgagaagtccaacggcaccatcatccacgtgaagggcaagcacctgtgtccttctccactgttccccggacctagcaagcctttctgggtgctcgttgttgttggcggcgtgctggcctgttactctctgctggttaccgtggccttcatcatcttttgggtccgaagcaagcggagcagaggcggccacagcgactacatgaacatgacccctagacggcccggaccaaccagaaagcactaccagccttacgctcctcctagagacttcgccgcctaccggtccagagtgaagttcagcagatccgccgatgctcccgcctatcagcagggacagaaccagctgtacaacgagctgaacctggggagaagagaagagtacgacgtgctggacaagcggagaggcagagatcctgagatgggcggcaagcccagacggaagaatcctcaagagggcctgtataatgagctgcagaaagacaagatggccgaggcctacagcgagatcggaatgaagggcgagcgcagaagaggcaagggacacgatggactgtaccagggcctgagcaccgccaccaaggatacctatgatgccctgcacatgcaggccctgcctccaagataa

SEQ ID NO: 52 - RNA, 747 nt, Synthetic construct
  source 1..747: mol_type = other RNA
atggctctgcctgtgacagctctgctgctgcctctggctctgcttctgcatgccgccagacctgactacaaggacgacgacgacaagatcgaagtgatgtaccctcctccttacctggacaacgagaagtccaacggcaccatcatccacgtgaagggcaagcacctgtgtccttctccactgttccccggacctagcaagcctttctgggtgctcgttgttgttggcggcgtgctggcctgttactctctgctggttaccgtggccttcatcatcttttgggtccgaagcaagcggagcagaggcggccacagcgactacatgaacatgacccctagacggcccggaccaaccagaaagcactaccagccttacgctcctcctagagacttcgccgcctaccggtccagagtgaagttcagcagatccgccgatgctcccgcctatcagcagggacagaaccagctgtacaacgagctgaacctggggagaagagaagagtacgacgtgctggacaagcggagaggcagagatcctgagatgggcggcaagcccagacggaagaatcctcaagagggcctgtataatgagctgcagaaagacaagatggccgaggcctacagcgagatcggaatgaagggcgagcgcagaagaggcaagggacacgatggactgtaccagggcctgagcaccgccaccaaggatacctatgatgccctgcacatgcaggccctgcctccaagataa

SEQ ID NO: 53 - DNA, 1473 bp, Synthetic construct
  source 1..1473: mol_type = other DNA
atggctctgcctgtgacagctctgctgctgcctctggctctgcttctgcatgccgccagacctgacatccagatgacacagagccctagcagcctgtctgccagcgtgggagacagagtgaccatcacctgtagagccagccagagcatcagctcctacctgaactggtatcagcagaagcccggcaaggcccctaagctgctgatctatgctgccagctctctgcagtctggcgtgcccagcagattttctggcagcggctctggcaccgacttcaccctgaccatatctagcctgcagcctgaggacttcgccacctactactgccagcagtcctacagcacccctcctacatttggccagggcaccaaggtggaaatcaaaggcggcggaggatctggcggaggtggaagtggcggaggcggatctgaagtgcagctggttgaatcaggtggcggcctggttcaacctggcggatctctgagactgagctgtgccgccagcggcttcaccttcagcgaccactatatggactgggtccgacaggcccctggcaaaggacttgagtgggtcggacggaccagaaacaaggccaacagctacaccacagagtacgccgcctctgtgaagggcagattcaccatcagccgggacgacagcaagaacagcctgtacctgcagatgaactccctgaaaaccgaggacaccgccgtgtactactgcgccagaggaatcagccccttctacttcgactattggggccagggaaccctcgtgaccgtttcttctgactacaaggacgacgacgacaagatcgaagtgatgtaccctcctccttacctggacaacgagaagtccaacggcaccatcatccacgtgaagggcaagcacctgtgtccttctccactgttccccggacctagcaagcctttctgggtgctcgttgttgttggcggcgtgctggcctgttactctctgctggttaccgtggccttcatcatcttttgggtccgaagcaagcggagcagaggcggccacagcgactacatgaacatgacccctagacggcccggaccaaccagaaagcactaccagccttacgctcctcctagagacttcgccgcctaccggtccagagtgaagttcagcagatccgccgatgctcccgcctatcagcagggacagaaccagctgtacaacgagctgaacctggggagaagagaagagtacgacgtgctggacaagcggagaggcagagatcctgagatgggcggcaagcccagacggaagaatcctcaagagggcctgtataatgagctgcagaaagacaagatggccgaggcctacagcgagatcggaatgaagggcgagcgcagaagaggcaagggacacgatggactgtaccagggcctgagcaccgccaccaaggatacctatgatgccctgcacatgcaggccctgcctccaagataa

SEQ ID NO: 54 - RNA, 1473 nt, Synthetic construct
  source 1..1473: mol_type = other RNA
atggctctgcctgtgacagctctgctgctgcctctggctctgcttctgcatgccgccagacctgacatccagatgacacagagccctagcagcctgtctgccagcgtgggagacagagtgaccatcacctgtagagccagccagagcatcagctcctacctgaactggtatcagcagaagcccggcaaggcccctaagctgctgatctatgctgccagctctctgcagtctggcgtgcccagcagattttctggcagcggctctggcaccgacttcaccctgaccatatctagcctgcagcctgaggacttcgccacctactactgccagcagtcctacagcacccctcctacatttggccagggcaccaaggtggaaatcaaaggcggcggaggatctggcggaggtggaagtggcggaggcggatctgaagtgcagctggttgaatcaggtggcggcctggttcaacctggcggatctctgagactgagctgtgccgccagcggcttcaccttcagcgaccactatatggactgggtccgacaggcccctggcaaaggacttgagtgggtcggacggaccagaaacaaggccaacagctacaccacagagtacgccgcctctgtgaagggcagattcaccatcagccgggacgacagcaagaacagcctgtacctgcagatgaactccctgaaaaccgaggacaccgccgtgtactactgcgccagaggaatcagccccttctacttcgactattggggccagggaaccctcgtgaccgtttcttctgactacaaggacgacgacgacaagatcgaagtgatgtaccctcctccttacctggacaacgagaagtccaacggcaccatcatccacgtgaagggcaagcacctgtgtccttctccactgttccccggacctagcaagcctttctgggtgctcgttgttgttggcggcgtgctggcctgttactctctgctggttaccgtggccttcatcatcttttgggtccgaagcaagcggagcagaggcggccacagcgactacatgaacatgacccctagacggcccggaccaaccagaaagcactaccagccttacgctcctcctagagacttcgccgcctaccggtccagagtgaagttcagcagatccgccgatgctcccgcctatcagcagggacagaaccagctgtacaacgagctgaacctggggagaagagaagagtacgacgtgctggacaagcggagaggcagagatcctgagatgggcggcaagcccagacggaagaatcctcaagagggcctgtataatgagctgcagaaagacaagatggccgaggcctacagcgagatcggaatgaagggcgagcgcagaagaggcaagggacacgatggactgtaccagggcctgagcaccgccaccaaggatacctatgatgccctgcacatgcaggccctgcctccaagataa

SEQ ID NO: 55 - DNA, 1488 bp, Synthetic construct
  source 1..1488: mol_type = other DNA
atggctctgcctgtgacagctctgctgctgcctctggctctgcttctgcatgccgccagacctgacatcgtgatgacacagagccctgacagcctggccgtgtctctgggagaaagagccaccatcaactgcaagagcagccagagcgtgctgtactccagcatcaacaagaactacctggcctggtatcagcagaagcccggccagcctcctaagctgctgatctactgggccagcaccagagaaagcggcgtgcccgatagattttctggcagcggctctggcaccgacttcaccctgacaattagctccctgcaggccgaggatgtggccgtgtactactgccagcagtactacagcaccccttacacctttggccagggcaccaaggtggaaatcaaaggcggcggaggatctggcggaggtggaagtggcggaggcggatctgaagttcagctggtgcagagcggcaccgaagtgaagaagcctggcgagagcctgaagatctcctgcaaaggctccggctacggcttcatcacctactggatcggctgggtccgacagatgcctggcaaaggccttgagtggatgggcatcatctaccccggcgacagcgagacaagatacagccctagcttccagggccaagtgaccatcagcgccgacaagagcatcaataccgcctacctgcagtggtccagcctgaaggcctctgacaccgccatctactattgtgccggcggaagcggcatcagcaccccaatggatgtttggggccagggaaccaccgtgaccgtttcttctgactacaaggacgacgacgacaagatcgaagtgatgtaccctcctccttacctggacaacgagaagtccaacggcaccatcatccacgtgaagggcaagcacctgtgtccttctccactgttccccggacctagcaagcctttctgggtgctcgttgttgttggcggcgtgctggcctgttactctctgctggttaccgtggccttcatcatcttttgggtccgaagcaagcggagcagaggcggccacagcgactacatgaacatgacccctagacggcccggaccaaccagaaagcactaccagccttacgctcctcctagagacttcgccgcctaccggtccagagtgaagttcagcagatccgccgatgctcccgcctatcagcagggacagaaccagctgtacaacgagctgaacctggggagaagagaagagtacgacgtgctggacaagcggagaggcagagatcctgagatgggcggcaagcccagacggaagaatcctcaagagggcctgtataatgagctgcagaaagacaagatggccgaggcctacagcgagatcggaatgaagggcgagcgcagaagaggcaagggacacgatggactgtaccagggcctgagcaccgccaccaaggatacctatgatgccctgcacatgcaggccctgcctccaagataa

SEQ ID NO: 56 - RNA, 1488 nt, Synthetic construct
  source 1..1488: mol_type = other RNA
atggctctgcctgtgacagctctgctgctgcctctggctctgcttctgcatgccgccagacctgacatcgtgatgacacagagccctgacagcctggccgtgtctctgggagaaagagccaccatcaactgcaagagcagccagagcgtgctgtactccagcatcaacaagaactacctggcctggtatcagcagaagcccggccagcctcctaagctgctgatctactgggccagcaccagagaaagcggcgtgcccgatagattttctggcagcggctctggcaccgacttcaccctgacaattagctccctgcaggccgaggatgtggccgtgtactactgccagcagtactacagcaccccttacacctttggccagggcaccaaggtggaaatcaaaggcggcggaggatctggcggaggtggaagtggcggaggcggatctgaagttcagctggtgcagagcggcaccgaagtgaagaagcctggcgagagcctgaagatctcctgcaaaggctccggctacggcttcatcacctactggatcggctgggtccgacagatgcctggcaaaggccttgagtggatgggcatcatctaccccggcgacagcgagacaagatacagccctagcttccagggccaagtgaccatcagcgccgacaagagcatcaataccgcctacctgcagtggtccagcctgaaggcctctgacaccgccatctactattgtgccggcggaagcggcatcagcaccccaatggatgtttggggccagggaaccaccgtgaccgtttcttctgactacaaggacgacgacgacaagatcgaagtgatgtaccctcctccttacctggacaacgagaagtccaacggcaccatcatccacgtgaagggcaagcacctgtgtccttctccactgttccccggacctagcaagcctttctgggtgctcgttgttgttggcggcgtgctggcctgttactctctgctggttaccgtggccttcatcatcttttgggtccgaagcaagcggagcagaggcggccacagcgactacatgaacatgacccctagacggcccggaccaaccagaaagcactaccagccttacgctcctcctagagacttcgccgcctaccggtccagagtgaagttcagcagatccgccgatgctcccgcctatcagcagggacagaaccagctgtacaacgagctgaacctggggagaagagaagagtacgacgtgctggacaagcggagaggcagagatcctgagatgggcggcaagcccagacggaagaatcctcaagagggcctgtataatgagctgcagaaagacaagatggccgaggcctacagcgagatcggaatgaagggcgagcgcagaagaggcaagggacacgatggactgtaccagggcctgagcaccgccaccaaggatacctatgatgccctgcacatgcaggccctgcctccaagataa

SEQ ID NO: 57 - DNA, 1512 bp, Synthetic construct
  source 1..1512: mol_type = other DNA
atggctctgcctgtgacagctctgctgctgcctctggctctgcttctgcatgccgccagacctgacatcgtgatgacacagagccctgacagcctggccgtgtctctgggagaaagagccaccatcaactgcaagagcagccagagcgtgctgtactccagcatcaacaagaactacctggcctggtatcagcagaagcccggccagcctcctaagctgctgatctactgggccagcaccagagaaagcggcgtgcccgatagattttctggcagcggctctggcaccgacttcaccctgacaattagctccctgcaggccgaggatgtggccgtgtactactgccagcagtactacagcaccccttacacctttggccagggcaccaaggtggaaatcaaaggcggcggaggatctggcggaggtggaagtggcggaggcggatctgaagttcagctggtgcagagcggcaccgaagtgaagaagcctggcgagagcctgaagatctcctgcaaaggctccggctacggcttcatcacctactggatcggctgggtccgacagatgcctggcaaaggccttgagtggatgggcatcatctaccccggcgacagcgagacaagatacagccctagcttccagggccaagtgaccatcagcgccgacaagagcatcaataccgcctacctgcagtggtccagcctgaaggcctctgacaccgccatctactattgtgccggcggaagcggcatcagcaccccaatggatgtttggggccagggaaccaccgtgaccgtttcttctgactacaaggacgacgacgacaagaagcccaccaccacaccagctcctagacctccaactcctgctcctacaatcgccagccagcctctgtctctgaggccagaagcttgtagacctgctgctggcggagccgtgcatacaagaggactggatttcgcctgcgacttctgggtgctcgttgttgttggcggcgtgctggcctgttactctctgctggttaccgtggccttcatcatcttttgggtccgaagcaagcggagcagaggcggccacagcgactacatgaacatgacccctagacggcccggaccaaccagaaagcactaccagccttacgctcctcctagagacttcgccgcctaccggtccagagtgaagttcagcagatccgccgatgctcccgcctatcagcagggacagaaccagctgtacaacgagctgaacctggggagaagagaagagtacgacgtgctggacaagcggagaggcagagatcctgagatgggcggcaagcccagacggaagaatcctcaagagggcctgtataatgagctgcagaaagacaagatggccgaggcctacagcgagatcggaatgaagggcgagcgcagaagaggcaagggacacgatggactgtaccagggcctgagcaccgccaccaaggatacctatgatgccctgcacatgcaggccctgcctccaagataa

SEQ ID NO: 58 - RNA, 1512 nt, Synthetic construct
  source 1..1512: mol_type = other RNA
atggctctgcctgtgacagctctgctgctgcctctggctctgcttctgcatgccgccagacctgacatcgtgatgacacagagccctgacagcctggccgtgtctctgggagaaagagccaccatcaactgcaagagcagccagagcgtgctgtactccagcatcaacaagaactacctggcctggtatcagcagaagcccggccagcctcctaagctgctgatctactgggccagcaccagagaaagcggcgtgcccgatagattttctggcagcggctctggcaccgacttcaccctgacaattagctccctgcaggccgaggatgtggccgtgtactactgccagcagtactacagcaccccttacacctttggccagggcaccaaggtggaaatcaaaggcggcggaggatctggcggaggtggaagtggcggaggcggatctgaagttcagctggtgcagagcggcaccgaagtgaagaagcctggcgagagcctgaagatctcctgcaaaggctccggctacggcttcatcacctactggatcggctgggtccgacagatgcctggcaaaggccttgagtggatgggcatcatctaccccggcgacagcgagacaagatacagccctagcttccagggccaagtgaccatcagcgccgacaagagcatcaataccgcctacctgcagtggtccagcctgaaggcctctgacaccgccatctactattgtgccggcggaagcggcatcagcaccccaatggatgtttggggccagggaaccaccgtgaccgtttcttctgactacaaggacgacgacgacaagaagcccaccaccacaccagctcctagacctccaactcctgctcctacaatcgccagccagcctctgtctctgaggccagaagcttgtagacctgctgctggcggagccgtgcatacaagaggactggatttcgcctgcgacttctgggtgctcgttgttgttggcggcgtgctggcctgttactctctgctggttaccgtggccttcatcatcttttgggtccgaagcaagcggagcagaggcggccacagcgactacatgaacatgacccctagacggcccggaccaaccagaaagcactaccagccttacgctcctcctagagacttcgccgcctaccggtccagagtgaagttcagcagatccgccgatgctcccgcctatcagcagggacagaaccagctgtacaacgagctgaacctggggagaagagaagagtacgacgtgctggacaagcggagaggcagagatcctgagatgggcggcaagcccagacggaagaatcctcaagagggcctgtataatgagctgcagaaagacaagatggccgaggcctacagcgagatcggaatgaagggcgagcgcagaagaggcaagggacacgatggactgtaccagggcctgagcaccgccaccaaggatacctatgatgccctgcacatgcaggccctgcctccaagataa

SEQ ID NO: 59 - DNA, 1728 bp, Synthetic construct
  source 1..1728: mol_type = other DNA
atggctctgcctgtgacagctctgctgctgcctctggctctgcttctgcatgccgccagacctgacatcgtgatgacacagagccctgacagcctggccgtgtctctgggagaaagagccaccatcaactgcaagagcagccagagcgtgctgtactccagcatcaacaagaactacctggcctggtatcagcagaagcccggccagcctcctaagctgctgatctactgggccagcaccagagaaagcggcgtgcccgatagattttctggcagcggctctggcaccgacttcaccctgacaattagctccctgcaggccgaggatgtggccgtgtactactgccagcagtactacagcaccccttacacctttggccagggcaccaaggtggaaatcaaaggcggcggaggatctggcggaggtggaagtggcggaggcggatctgaagttcagctggtgcagagcggcaccgaagtgaagaagcctggcgagagcctgaagatctcctgcaaaggctccggctacggcttcatcacctactggatcggctgggtccgacagatgcctggcaaaggccttgagtggatgggcatcatctaccccggcgacagcgagacaagatacagccctagcttccagggccaagtgaccatcagcgccgacaagagcatcaataccgcctacctgcagtggtccagcctgaaggcctctgacaccgccatctactattgtgccggcggaagcggcatcagcaccccaatggatgtttggggccagggaaccaccgtgaccgtttcttctgactacaaggacgacgacgacaaggaatctaagtacggccctccttgtcctccatgtcctggccagccaagagaaccccaggtgtacacactgcctccaagccaagaggaaatgaccaagaaccaggtgtccctgacctgcctggtcaagggcttctacccttccgatatcgccgtggaatgggagagcaatggccagcctgagaacaactacaagaccacacctcctgtgctggacagcgacggctcattcttcctgtacagcagactgaccgtggacaagagcagatggcaagagggcaacgtgttcagctgcagcgtgatgcacgaggccctgcacaaccactacacccagaagtctctgagcctgagcctgggcaagttctgggtgctcgttgttgttggcggcgtgctggcctgttactctctgctggttaccgtggccttcatcatcttttgggtccgaagcaagcggagcagaggcggccacagcgactacatgaacatgacccctagacggcccggaccaaccagaaagcactaccagccttacgctcctcctagagacttcgccgcctaccggtccagagtgaagttcagcagatccgccgatgctcccgcctatcagcagggacagaaccagctgtacaacgagctgaacctggggagaagagaagagtacgacgtgctggacaagcggagaggcagagatcctgagatgggcggcaagcccagacggaagaatcctcaagagggcctgtataatgagctgcagaaagacaagatggccgaggcctacagcgagatcggaatgaagggcgagcgcagaagaggcaagggacacgatggactgtaccagggcctgagcaccgccaccaaggatacctatgatgccctgcacatgcaggccctgcctccaagataa

SEQ ID NO: 60 - RNA, 1728 nt, Synthetic construct
  source 1..1728: mol_type = other RNA
atggctctgcctgtgacagctctgctgctgcctctggctctgcttctgcatgccgccagacctgacatcgtgatgacacagagccctgacagcctggccgtgtctctgggagaaagagccaccatcaactgcaagagcagccagagcgtgctgtactccagcatcaacaagaactacctggcctggtatcagcagaagcccggccagcctcctaagctgctgatctactgggccagcaccagagaaagcggcgtgcccgatagattttctggcagcggctctggcaccgacttcaccctgacaattagctccctgcaggccgaggatgtggccgtgtactactgccagcagtactacagcaccccttacacctttggccagggcaccaaggtggaaatcaaaggcggcggaggatctggcggaggtggaagtggcggaggcggatctgaagttcagctggtgcagagcggcaccgaagtgaagaagcctggcgagagcctgaagatctcctgcaaaggctccggctacggcttcatcacctactggatcggctgggtccgacagatgcctggcaaaggccttgagtggatgggcatcatctaccccggcgacagcgagacaagatacagccctagcttccagggccaagtgaccatcagcgccgacaagagcatcaataccgcctacctgcagtggtccagcctgaaggcctctgacaccgccatctactattgtgccggcggaagcggcatcagcaccccaatggatgtttggggccagggaaccaccgtgaccgtttcttctgactacaaggacgacgacgacaaggaatctaagtacggccctccttgtcctccatgtcctggccagccaagagaaccccaggtgtacacactgcctccaagccaagaggaaatgaccaagaaccaggtgtccctgacctgcctggtcaagggcttctacccttccgatatcgccgtggaatgggagagcaatggccagcctgagaacaactacaagaccacacctcctgtgctggacagcgacggctcattcttcctgtacagcagactgaccgtggacaagagcagatggcaagagggcaacgtgttcagctgcagcgtgatgcacgaggccctgcacaaccactacacccagaagtctctgagcctgagcctgggcaagttctgggtgctcgttgttgttggcggcgtgctggcctgttactctctgctggttaccgtggccttcatcatcttttgggtccgaagcaagcggagcagaggcggccacagcgactacatgaacatgacccctagacggcccggaccaaccagaaagcactaccagccttacgctcctcctagagacttcgccgcctaccggtccagagtgaagttcagcagatccgccgatgctcccgcctatcagcagggacagaaccagctgtacaacgagctgaacctggggagaagagaagagtacgacgtgctggacaagcggagaggcagagatcctgagatgggcggcaagcccagacggaagaatcctcaagagggcctgtataatgagctgcagaaagacaagatggccgaggcctacagcgagatcggaatgaagggcgagcgcagaagaggcaagggacacgatggactgtaccagggcctgagcaccgccaccaaggatacctatgatgccctgcacatgcaggccctgcctccaagataa

SEQ ID NO: 61 - DNA, 2058 bp, Synthetic construct
  source 1..2058: mol_type = other DNA
atggctctgcctgtgacagctctgctgctgcctctggctctgcttctgcatgccgccagacctgacatcgtgatgacacagagccctgacagcctggccgtgtctctgggagaaagagccaccatcaactgcaagagcagccagagcgtgctgtactccagcatcaacaagaactacctggcctggtatcagcagaagcccggccagcctcctaagctgctgatctactgggccagcaccagagaaagcggcgtgcccgatagattttctggcagcggctctggcaccgacttcaccctgacaattagctccctgcaggccgaggatgtggccgtgtactactgccagcagtactacagcaccccttacacctttggccagggcaccaaggtggaaatcaaaggcggcggaggatctggcggaggtggaagtggcggaggcggatctgaagttcagctggtgcagagcggcaccgaagtgaagaagcctggcgagagcctgaagatctcctgcaaaggctccggctacggcttcatcacctactggatcggctgggtccgacagatgcctggcaaaggccttgagtggatgggcatcatctaccccggcgacagcgagacaagatacagccctagcttccagggccaagtgaccatcagcgccgacaagagcatcaataccgcctacctgcagtggtccagcctgaaggcctctgacaccgccatctactattgtgccggcggaagcggcatcagcaccccaatggatgtttggggccagggaaccaccgtgaccgtttcttctgactacaaggacgacgacgacaaggaatctaagtacggccctccttgtcctccatgtcctgctccagagtttctcggcggaccctccgtgttcctgtttcctccaaagcctaaggacaccctgatgatcagcagaacccctgaagtgacctgcgtggtggtggacgtttcccaagaggaccctgaggtgcagttcaattggtacgtggacggcgtggaagtgcacaacgccaagaccaagcctagagaggaacagttcaacagcacctacagagtggtgtccgtgctgaccgtgctgcaccaggattggctgaacggcaaagagtacaagtgcaaggtgtccaacaagggcctgcctagcagcatcgagaaaaccatcagcaaggccaagggccagccaagagaaccccaggtgtacacactgcctccaagccaagaggaaatgaccaagaaccaggtgtccctgacctgcctggtcaagggcttctacccttccgatatcgccgtggaatgggagagcaatggccagcctgagaacaactacaagaccacacctcctgtgctggacagcgacggctcattcttcctgtacagcagactgaccgtggacaagagcagatggcaagagggcaacgtgttcagctgcagcgtgatgcacgaggccctgcacaaccactacacccagaagtctctgagcctgagcctgggcaagttctgggtgctcgttgttgttggcggcgtgctggcctgttactctctgctggttaccgtggccttcatcatcttttgggtccgaagcaagcggagcagaggcggccacagcgactacatgaacatgacccctagacggcccggaccaaccagaaagcactaccagccttacgctcctcctagagacttcgccgcctaccggtccagagtgaagttcagcagatccgccgatgctcccgcctatcagcagggacagaaccagctgtacaacgagctgaacctggggagaagagaagagtacgacgtgctggacaagcggagaggcagagatcctgagatgggcggcaagcccagacggaagaatcctcaagagggcctgtataatgagctgcagaaagacaagatggccgaggcctacagcgagatcggaatgaagggcgagcgcagaagaggcaagggacacgatggactgtaccagggcctgagcaccgccaccaaggatacctatgatgccctgcacatgcaggccctgcctccaagataa

SEQ ID NO: 62 - RNA, 2058 nt, Synthetic construct
  source 1..2058: mol_type = other RNA
atggctctgcctgtgacagctctgctgctgcctctggctctgcttctgcatgccgccagacctgacatcgtgatgacacagagccctgacagcctggccgtgtctctgggagaaagagccaccatcaactgcaagagcagccagagcgtgctgtactccagcatcaacaagaactacctggcctggtatcagcagaagcccggccagcctcctaagctgctgatctactgggccagcaccagagaaagcggcgtgcccgatagattttctggcagcggctctggcaccgacttcaccctgacaattagctccctgcaggccgaggatgtggccgtgtactactgccagcagtactacagcaccccttacacctttggccagggcaccaaggtggaaatcaaaggcggcggaggatctggcggaggtggaagtggcggaggcggatctgaagttcagctggtgcagagcggcaccgaagtgaagaagcctggcgagagcctgaagatctcctgcaaaggctccggctacggcttcatcacctactggatcggctgggtccgacagatgcctggcaaaggccttgagtggatgggcatcatctaccccggcgacagcgagacaagatacagccctagcttccagggccaagtgaccatcagcgccgacaagagcatcaataccgcctacctgcagtggtccagcctgaaggcctctgacaccgccatctactattgtgccggcggaagcggcatcagcaccccaatggatgtttggggccagggaaccaccgtgaccgtttcttctgactacaaggacgacgacgacaaggaatctaagtacggccctccttgtcctccatgtcctgctccagagtttctcggcggaccctccgtgttcctgtttcctccaaagcctaaggacaccctgatgatcagcagaacccctgaagtgacctgcgtggtggtggacgtttcccaagaggaccctgaggtgcagttcaattggtacgtggacggcgtggaagtgcacaacgccaagaccaagcctagagaggaacagttcaacagcacctacagagtggtgtccgtgctgaccgtgctgcaccaggattggctgaacggcaaagagtacaagtgcaaggtgtccaacaagggcctgcctagcagcatcgagaaaaccatcagcaaggccaagggccagccaagagaaccccaggtgtacacactgcctccaagccaagaggaaatgaccaagaaccaggtgtccctgacctgcctggtcaagggcttctacccttccgatatcgccgtggaatgggagagcaatggccagcctgagaacaactacaagaccacacctcctgtgctggacagcgacggctcattcttcctgtacagcagactgaccgtggacaagagcagatggcaagagggcaacgtgttcagctgcagcgtgatgcacgaggccctgcacaaccactacacccagaagtctctgagcctgagcctgggcaagttctgggtgctcgttgttgttggcggcgtgctggcctgttactctctgctggttaccgtggccttcatcatcttttgggtccgaagcaagcggagcagaggcggccacagcgactacatgaacatgacccctagacggcccggaccaaccagaaagcactaccagccttacgctcctcctagagacttcgccgcctaccggtccagagtgaagttcagcagatccgccgatgctcccgcctatcagcagggacagaaccagctgtacaacgagctgaacctggggagaagagaagagtacgacgtgctggacaagcggagaggcagagatcctgagatgggcggcaagcccagacggaagaatcctcaagagggcctgtataatgagctgcagaaagacaagatggccgaggcctacagcgagatcggaatgaagggcgagcgcagaagaggcaagggacacgatggactgtaccagggcctgagcaccgccaccaaggatacctatgatgccctgcacatgcaggccctgcctccaagataa

SEQ ID NO: 63 - DNA, 2037 bp, Synthetic construct
  source 1..2037: mol_type = other DNA
atggctctgcctgttacagctctgctgctgcctctggctctgcttctgcatgctgctagacctcaggtgcagctggtggaatctggtggcggagttgtgcagcctggcagaagcctgagactgtcttgtgccgccagcggcttcacctttagcagctatgccatgcactgggtccgacaggcccctggcaaaggacttgaatgggtcgccgtgattcccttcgacggccggaacaagtactacgccgatagcgtgaccggcagattcaccatcagccgggacaacagcaagaacaccctgtacctgcagatgaacagcctgagagccgaggacaccgccgtgtactactgtgcctctagcagcggctacctgttccacagcgattattggggccagggcaccctggtcacagtttctagcggaggcggaggaagtggcggcggaggatctggcggtggtggttctgatatccagatgacacagagccccagcacactgtctgccagcgtgggagacagagtgaccatcacctgtagagccagccagagcatcagcaactggctggcctggttccagcagaagccaggcaaagcccctaagctgctgatctacgaggccagctctctggaaagcggcgtgccaagcagattttctggcagcggctctggcaccgagttcaccctgaccatcagtagcctgcagcctgacgacttcgccacctactactgccagcagtacaacagctacccctggacctttggacagggcaccaaggtggaaatcaaggactacaaggacgacgacgacaaggaatctaagtacggccctccttgtcctccatgtcctgctccacctgtggccggaccctccgtgttcctgtttcctccaaagcctaaggacaccctgatgatcagcagaacccctgaagtgacctgcgtggtggtggacgtttcccaagaggaccctgaggtgcagttcaattggtacgtggacggcgtggaagtgcacaacgccaagaccaagcctagagaggaacagttccagagcacctacagagtggtgtccgtgctgaccgtgctgcaccaggattggctgaacggcaaagagtacaagtgcaaggtgtccaacaagggcctgcctagcagcatcgagaaaaccatcagcaaggccaagggccagccaagagaaccccaggtgtacacactgcctccaagccaagaggaaatgaccaagaaccaggtgtccctgacctgcctggtcaagggcttctacccttccgatatcgccgtggaatgggagagcaatggccagcctgagaacaactacaagaccacacctcctgtgctggacagcgacggctcattcttcctgtacagcagactgaccgtggacaagagcagatggcaagagggcaacgtgttcagctgcagcgtgatgcacgaggccctgcacaaccactacacccagaagtctctgagcctgagcctgggcaagttctgggtgctcgttgttgttggcggcgtgctggcctgttactctctgctggttaccgtggccttcatcatcttttgggtccgaagcaagcggagcagaggcggccacagcgactacatgaacatgacccctagacggcccggaccaaccagaaagcactaccagccttacgctcctcctagagacttcgccgcctaccggtccagagtgaagttcagcagatccgccgatgctcccgcctatcagcagggacagaaccagctgtacaacgagctgaacctggggagaagagaagagtacgacgtgctggacaagcggagaggcagagatcctgagatgggcggcaagcccagacggaagaatcctcaagagggcctgtataatgagctgcagaaagacaagatggccgaggcctacagcgagatcggaatgaagggcgagcgcagaagaggcaagggacacgatggactgtaccagggcctgagcaccgccaccaaggatacctatgatgccctgcacatgcaggccctgcctccaagataa

SEQ ID NO: 64 - RNA, 2037 nt, Synthetic construct
  source 1..2037: mol_type = other RNA
atggctctgcctgttacagctctgctgctgcctctggctctgcttctgcatgctgctagacctcaggtgcagctggtggaatctggtggcggagttgtgcagcctggcagaagcctgagactgtcttgtgccgccagcggcttcacctttagcagctatgccatgcactgggtccgacaggcccctggcaaaggacttgaatgggtcgccgtgattcccttcgacggccggaacaagtactacgccgatagcgtgaccggcagattcaccatcagccgggacaacagcaagaacaccctgtacctgcagatgaacagcctgagagccgaggacaccgccgtgtactactgtgcctctagcagcggctacctgttccacagcgattattggggccagggcaccctggtcacagtttctagcggaggcggaggaagtggcggcggaggatctggcggtggtggttctgatatccagatgacacagagccccagcacactgtctgccagcgtgggagacagagtgaccatcacctgtagagccagccagagcatcagcaactggctggcctggttccagcagaagccaggcaaagcccctaagctgctgatctacgaggccagctctctggaaagcggcgtgccaagcagattttctggcagcggctctggcaccgagttcaccctgaccatcagtagcctgcagcctgacgacttcgccacctactactgccagcagtacaacagctacccctggacctttggacagggcaccaaggtggaaatcaaggactacaaggacgacgacgacaaggaatctaagtacggccctccttgtcctccatgtcctgctccacctgtggccggaccctccgtgttcctgtttcctccaaagcctaaggacaccctgatgatcagcagaacccctgaagtgacctgcgtggtggtggacgtttcccaagaggaccctgaggtgcagttcaattggtacgtggacggcgtggaagtgcacaacgccaagaccaagcctagagaggaacagttccagagcacctacagagtggtgtccgtgctgaccgtgctgcaccaggattggctgaacggcaaagagtacaagtgcaaggtgtccaacaagggcctgcctagcagcatcgagaaaaccatcagcaaggccaagggccagccaagagaaccccaggtgtacacactgcctccaagccaagaggaaatgaccaagaaccaggtgtccctgacctgcctggtcaagggcttctacccttccgatatcgccgtggaatgggagagcaatggccagcctgagaacaactacaagaccacacctcctgtgctggacagcgacggctcattcttcctgtacagcagactgaccgtggacaagagcagatggcaagagggcaacgtgttcagctgcagcgtgatgcacgaggccctgcacaaccactacacccagaagtctctgagcctgagcctgggcaagttctgggtgctcgttgttgttggcggcgtgctggcctgttactctctgctggttaccgtggccttcatcatcttttgggtccgaagcaagcggagcagaggcggccacagcgactacatgaacatgacccctagacggcccggaccaaccagaaagcactaccagccttacgctcctcctagagacttcgccgcctaccggtccagagtgaagttcagcagatccgccgatgctcccgcctatcagcagggacagaaccagctgtacaacgagctgaacctggggagaagagaagagtacgacgtgctggacaagcggagaggcagagatcctgagatgggcggcaagcccagacggaagaatcctcaagagggcctgtataatgagctgcagaaagacaagatggccgaggcctacagcgagatcggaatgaagggcgagcgcagaagaggcaagggacacgatggactgtaccagggcctgagcaccgccaccaaggatacctatgatgccctgcacatgcaggccctgcctccaagataa

SEQ ID NO: 65 - DNA, 2049 bp, Synthetic construct
  source 1..2049: mol_type = other DNA
atggctctgcctgttacagctctgctgctgcctctggctctgcttctgcatgctgctagacctcaggtgcagctggttcagtctggcgccgaagtgaagaaacctggcgcctctgtgaaggtgtcctgcaaggccagcggctacccttttaccagctacggcatcagctgggtccgacaggctcctggacaaggcttggaatggatgggctggatcagcacctacaacggcaacaccaactacgcccagaaattccagggcagagtgaccatgaccaccgacaccagcaccaccaccggctacatggaactgcggagactgagaagcgacgacaccgccgtgtactactgcgccagagattacaccagaggcgcttggtttggcgagtctctgatcggcggcttcgacaattggggccagggaacactggtcaccgtttctagcggaggcggaggatctggtggcggaggaagtggcggaggcggttctgaaattgtgctgacacagagccccggcacactgtcactttctccaggcgaaagagccacactgagctgtagagccagccagaccgtgtctagcacaagcctggcttggtatcagcagaagcctggacaggcccctcggctgttgatctacggtgcttctagccgcgccacaggcatccccgatagattttctggcagcggctccggcaccgacttcaccctgacaatcagcagactggaacccgaggacttcgccgtgtattattgccagcagcacgataccagcctgacctttggcggcggaacaaaggtggaaatcaaggactacaaggacgacgacgacaaggaatctaagtacggccctccttgtcctccatgtcctgctccacctgtggccggaccctccgtgttcctgtttcctccaaagcctaaggacaccctgatgatcagcagaacccctgaagtgacctgcgtggtggtggacgtttcccaagaggaccctgaggtgcagttcaattggtacgtggacggcgtggaagtgcacaacgccaagaccaagcctagagaggaacagttccagagcacctacagagtggtgtccgtgctgaccgtgctgcaccaggattggctgaacggcaaagagtacaagtgcaaggtgtccaacaagggcctgcctagcagcatcgagaaaaccatcagcaaggccaagggccagccaagagaaccccaggtgtacacactgcctccaagccaagaggaaatgaccaagaaccaggtgtccctgacctgcctggtcaagggcttctacccttccgatatcgccgtggaatgggagagcaatggccagcctgagaacaactacaagaccacacctcctgtgctggacagcgacggctcattcttcctgtacagcagactgaccgtggacaagagcagatggcaagagggcaacgtgttcagctgcagcgtgatgcacgaggccctgcacaaccactacacccagaagtctctgagcctgagcctgggcaagttctgggtgctcgttgttgttggcggcgtgctggcctgttactctctgctggttaccgtggccttcatcatcttttgggtccgaagcaagcggagcagaggcggccacagcgactacatgaacatgacccctagacggcccggaccaaccagaaagcactaccagccttacgctcctcctagagacttcgccgcctaccggtccagagtgaagttcagcagatccgccgatgctcccgcctatcagcagggacagaaccagctgtacaacgagctgaacctggggagaagagaagagtacgacgtgctggacaagcggagaggcagagatcctgagatgggcggcaagcccagacggaagaatcctcaagagggcctgtataatgagctgcagaaagacaagatggccgaggcctacagcgagatcggaatgaagggcgagcgcagaagaggcaagggacacgatggactgtaccagggcctgagcaccgccaccaaggatacctatgatgccctgcacatgcaggccctg

SEQ ID NO: 66 - RNA, 2049 nt, Synthetic construct
  source 1..2049: mol_type = other RNA
atggctctgcctgttacagctctgctgctgcctctggctctgcttctgcatgctgctagacctcaggtgcagctggttcagtctggcgccgaagtgaagaaacctggcgcctctgtgaaggtgtcctgcaaggccagcggctacccttttaccagctacggcatcagctgggtccgacaggctcctggacaaggcttggaatggatgggctggatcagcacctacaacggcaacaccaactacgcccagaaattccagggcagagtgaccatgaccaccgacaccagcaccaccaccggctacatggaactgcggagactgagaagcgacgacaccgccgtgtactactgcgccagagattacaccagaggcgcttggtttggcgagtctctgatcggcggcttcgacaattggggccagggaacactggtcaccgtttctagcggaggcggaggatctggtggcggaggaagtggcggaggcggttctgaaattgtgctgacacagagccccggcacactgtcactttctccaggcgaaagagccacactgagctgtagagccagccagaccgtgtctagcacaagcctggcttggtatcagcagaagcctggacaggcccctcggctgttgatctacggtgcttctagccgcgccacaggcatccccgatagattttctggcagcggctccggcaccgacttcaccctgacaatcagcagactggaacccgaggacttcgccgtgtattattgccagcagcacgataccagcctgacctttggcggcggaacaaaggtggaaatcaaggactacaaggacgacgacgacaaggaatctaagtacggccctccttgtcctccatgtcctgctccacctgtggccggaccctccgtgttcctgtttcctccaaagcctaaggacaccctgatgatcagcagaacccctgaagtgacctgcgtggtggtggacgtttcccaagaggaccctgaggtgcagttcaattggtacgtggacggcgtggaagtgcacaacgccaagaccaagcctagagaggaacagttccagagcacctacagagtggtgtccgtgctgaccgtgctgcaccaggattggctgaacggcaaagagtacaagtgcaaggtgtccaacaagggcctgcctagcagcatcgagaaaaccatcagcaaggccaagggccagccaagagaaccccaggtgtacacactgcctccaagccaagaggaaatgaccaagaaccaggtgtccctgacctgcctggtcaagggcttctacccttccgatatcgccgtggaatgggagagcaatggccagcctgagaacaactacaagaccacacctcctgtgctggacagcgacggctcattcttcctgtacagcagactgaccgtggacaagagcagatggcaagagggcaacgtgttcagctgcagcgtgatgcacgaggccctgcacaaccactacacccagaagtctctgagcctgagcctgggcaagttctgggtgctcgttgttgttggcggcgtgctggcctgttactctctgctggttaccgtggccttcatcatcttttgggtccgaagcaagcggagcagaggcggccacagcgactacatgaacatgacccctagacggcccggaccaaccagaaagcactaccagccttacgctcctcctagagacttcgccgcctaccggtccagagtgaagttcagcagatccgccgatgctcccgcctatcagcagggacagaaccagctgtacaacgagctgaacctggggagaagagaagagtacgacgtgctggacaagcggagaggcagagatcctgagatgggcggcaagcccagacggaagaatcctcaagagggcctgtataatgagctgcagaaagacaagatggccgaggcctacagcgagatcggaatgaagggcgagcgcagaagaggcaagggacacgatggactgtaccagggcctgagcaccgccaccaaggatacctatgatgccctgcacatgcaggccctg

SEQ ID NO: 67 - DNA, 2079 bp, Synthetic construct
  source 1..2079: mol_type = other DNA
atggctctgcctgttacagctctgctgctgcctctggctctgcttctgcatgccgctagacctgaggtgcagctggttgaatctggcgccgaagtgaagaaaccaggcgcctctgtgaaggtgtcctgcaaggtgtccggctacaccctgacagagctgagcatgcactgggtccgacaggcccctggaaaaggccttgaatggatgggcggcttcgaccccgaagatggcgagactatgtacgcccagaaattccagggcagagtgaccatgaccgaggacaccagcaccgacaccgcctacatggaactgagcagcctgagaagcgaggataccgccgtgtactactgcgccacatctacagccgtggccggcacacctgacctgttcgattactactacggcatggacgtgtggggccagggcacaacagtgacagtttcttctggcggcggaggatctggcggaggtggaagcggaggcggtggatctgagatcgtgatgacacagagccctctgtctagccccgtgacactgggacagcctgccagcatcagctgtagaagcagccagagcctggtgcacagcgacggcaatacctacctgtcttggctgcagcagaggcctggacagcctcctagactgctgatctacaagatcagcaaccggttcagcggcgtgcccgatagattttctggtagcggagccggcaccgacttcaccctgaagatcagtagagtggaagccgaggacgtgggcgtgtactattgcacacaggccacacagttcccttacaccttcggacagggcaccaaggtggacatcaaggactacaaggacgacgacgacaaggaatctaagtacggccctccttgtcctccatgtcctgctccacctgtggccggaccctccgtgttcctgtttcctccaaagcctaaggacaccctgatgatcagcagaacccctgaagtgacctgcgtggtggtggacgtttcccaagaggaccctgaggtgcagttcaattggtacgtggacggcgtggaagtgcacaacgccaagaccaagcctagagaggaacagttccagagcacctacagagtggtgtccgtgctgaccgtgctgcaccaggattggctgaacggcaaagagtacaagtgcaaggtgtccaacaagggcctgcctagcagcatcgagaaaaccatcagcaaggccaagggccagccaagagaaccccaggtgtacacactgcctccaagccaagaggaaatgaccaagaaccaggtgtccctgacctgcctggtcaagggcttctacccttccgatatcgccgtggaatgggagagcaatggccagcctgagaacaactacaagaccacacctcctgtgctggacagcgacggctcattcttcctgtacagcagactgaccgtggacaagagcagatggcaagagggcaacgtgttcagctgcagcgtgatgcacgaggccctgcacaaccactacacccagaagtctctgagcctgagcctgggcaagttctgggtgctcgttgttgttggcggcgtgctggcctgttactctctgctggttaccgtggccttcatcatcttttgggtccgaagcaagcggagcagaggcggccacagcgactacatgaacatgacccctagacggcccggaccaaccagaaagcactaccagccttacgctcctcctagagacttcgccgcctaccggtccagagtgaagttcagcagatccgccgatgctcccgcctatcagcagggacagaaccagctgtacaacgagctgaacctggggagaagagaagagtacgacgtgctggacaagcggagaggcagagatcctgagatgggcggcaagcccagacggaagaatcctcaagagggcctgtataatgagctgcagaaagacaagatggccgaggcctacagcgagatcggaatgaagggcgagcgcagaagaggcaagggacacgatggactgtaccagggcctgagcaccgccaccaaggatacctatgatgccctgcacatgcaggccctgcctccaagataa

SEQ ID NO: 68 - RNA, 2079 nt, Synthetic construct
  source 1..2079: mol_type = other RNA
atggctctgcctgttacagctctgctgctgcctctggctctgcttctgcatgccgctagacctgaggtgcagctggttgaatctggcgccgaagtgaagaaaccaggcgcctctgtgaaggtgtcctgcaaggtgtccggctacaccctgacagagctgagcatgcactgggtccgacaggcccctggaaaaggccttgaatggatgggcggcttcgaccccgaagatggcgagactatgtacgcccagaaattccagggcagagtgaccatgaccgaggacaccagcaccgacaccgcctacatggaactgagcagcctgagaagcgaggataccgccgtgtactactgcgccacatctacagccgtggccggcacacctgacctgttcgattactactacggcatggacgtgtggggccagggcacaacagtgacagtttcttctggcggcggaggatctggcggaggtggaagcggaggcggtggatctgagatcgtgatgacacagagccctctgtctagccccgtgacactgggacagcctgccagcatcagctgtagaagcagccagagcctggtgcacagcgacggcaatacctacctgtcttggctgcagcagaggcctggacagcctcctagactgctgatctacaagatcagcaaccggttcagcggcgtgcccgatagattttctggtagcggagccggcaccgacttcaccctgaagatcagtagagtggaagccgaggacgtgggcgtgtactattgcacacaggccacacagttcccttacaccttcggacagggcaccaaggtggacatcaaggactacaaggacgacgacgacaaggaatctaagtacggccctccttgtcctccatgtcctgctccacctgtggccggaccctccgtgttcctgtttcctccaaagcctaaggacaccctgatgatcagcagaacccctgaagtgacctgcgtggtggtggacgtttcccaagaggaccctgaggtgcagttcaattggtacgtggacggcgtggaagtgcacaacgccaagaccaagcctagagaggaacagttccagagcacctacagagtggtgtccgtgctgaccgtgctgcaccaggattggctgaacggcaaagagtacaagtgcaaggtgtccaacaagggcctgcctagcagcatcgagaaaaccatcagcaaggccaagggccagccaagagaaccccaggtgtacacactgcctccaagccaagaggaaatgaccaagaaccaggtgtccctgacctgcctggtcaagggcttctacccttccgatatcgccgtggaatgggagagcaatggccagcctgagaacaactacaagaccacacctcctgtgctggacagcgacggctcattcttcctgtacagcagactgaccgtggacaagagcagatggcaagagggcaacgtgttcagctgcagcgtgatgcacgaggccctgcacaaccactacacccagaagtctctgagcctgagcctgggcaagttctgggtgctcgttgttgttggcggcgtgctggcctgttactctctgctggttaccgtggccttcatcatcttttgggtccgaagcaagcggagcagaggcggccacagcgactacatgaacatgacccctagacggcccggaccaaccagaaagcactaccagccttacgctcctcctagagacttcgccgcctaccggtccagagtgaagttcagcagatccgccgatgctcccgcctatcagcagggacagaaccagctgtacaacgagctgaacctggggagaagagaagagtacgacgtgctggacaagcggagaggcagagatcctgagatgggcggcaagcccagacggaagaatcctcaagagggcctgtataatgagctgcagaaagacaagatggccgaggcctacagcgagatcggaatgaagggcgagcgcagaagaggcaagggacacgatggactgtaccagggcctgagcaccgccaccaaggatacctatgatgccctgcacatgcaggccctgcctccaagataa

SEQ ID NO: 69 - DNA, 2910 bp, Synthetic construct
  source 1..2910: mol_type = other DNA
atggctctgcctgttacagctctgctgctgcctctggctctgcttctgcatgccgctagacctgaggtgcagctggttgaatctggcgccgaagtgaagaaaccaggcgcctctgtgaaggtgtcctgcaaggtgtccggctacaccctgacagagctgagcatgcactgggtccgacaggcccctggaaaaggccttgaatggatgggcggcttcgaccccgaagatggcgagactatgtacgcccagaaattccagggcagagtgaccatgaccgaggacaccagcaccgacaccgcctacatggaactgagcagcctgagaagcgaggataccgccgtgtactactgcgccacatctacagccgtggccggcacacctgacctgttcgattactactacggcatggacgtgtggggccagggcacaacagtgacagtttcttctggcggcggaggatctggcggaggtggaagcggaggcggtggatctgagatcgtgatgacacagagccctctgtctagccccgtgacactgggacagcctgccagcatcagctgtagaagcagccagagcctggtgcacagcgacggcaatacctacctgtcttggctgcagcagaggcctggacagcctcctagactgctgatctacaagatcagcaaccggttcagcggcgtgcccgatagattttctggtagcggagccggcaccgacttcaccctgaagatcagtagagtggaagccgaggacgtgggcgtgtactattgcacacaggccacacagttcccttacaccttcggacagggcaccaaggtggacatcaaggactacaaggacgacgacgacaagcagctttcattaccctctatccttccaaatgaaaatgaaaaggttgtgcagctgaattcatccttttctctgagatgctttggggagagtgaagtgagctggcagtaccccatgtctgaagaagagagctccgatgtggaaatcagaaatgaagaaaacaacagcggcctttttgtgacggtcttggaagtgagcagtgcctcggcggcccacacagggttgtacacttgctattacaaccacactcagacagaagagaatgagcttgaaggcaggcacatttacatctatgtgccagacccagatgtagcctttgtacctctaggaatgacggattatttagtcatcgtggaggatgatgattctgccattataccttgtcgcacaactgatcccgagactcctgtaaccttacacaacagtgagggggtggtacctgcctcctacgacagcagacagggctttaatgggaccttcactgtagggccctatatctgtgaggccaccgtcaaaggaaagaagttccagaccatcccatttaatgtttatgctttaaaagcaacatcagagctggatctagaaatggaagctcttaaaaccgtgtataagtcaggggaaacgattgtggtcacctgtgctgtttttaacaatgaggtggttgaccttcaatggacttaccctggagaagtgaaaggcaaaggcatcacaatgctggaagaaatcaaagtcccatccatcaaattggtgtacactttgacggtccccgaggccacggtgaaagacagtggagattacgaatgtgctgcccgccaggctaccagggaggtcaaagaaatgaagaaagtcactatttctgtccatgagaaaggtttcattgaaatcaaacccaccttcagccagttggaagctgtcaacctgcatgaagtcaaacattttgttgtagaggtgcgggcctacccacctcccaggatatcctggctgaaaaacaatctgactctgattgaaaatctcactgagatcaccactgatgtggaaaagattcaggaaataaggtatcgaagcaaattaaagctgatccgtgctaaggaagaagacagtggccattatactattgtagctcaaaatgaagatgctgtgaagagctatacttttgaactgttaactcaagttccttcatccattctggacttggtcgatgatcaccatggctcaactgggggacagacggtgaggtgcacagctgaaggcacgccgcttcctgatattgagtggatgatatgcaaagatattaagaaatgtaataatgaaacttcctggactattttggccaacaatgtctcaaacatcatcacggagatccactcccgagacaggagtaccgtggagggccgtgtgactttcgccaaagtggaggagaccatcgccgtgcgatgcctggctaagaatctccttggagctgagaaccgagagctgaagctggtggctcccaccctgcgttctgaactcacggtggctttctgggtgctcgttgttgttggcggcgtgctggcctgttactctctgctggttaccgtggccttcatcatcttttgggtccgaagcaagcggagcagaggcggccacagcgactacatgaacatgacccctagacggcccggaccaaccagaaagcactaccagccttacgctcctcctagagacttcgccgcctaccggtccagagtgaagttcagcagatccgccgatgctcccgcctatcagcagggacagaaccagctgtacaacgagctgaacctggggagaagagaagagtacgacgtgctggacaagcggagaggcagagatcctgagatgggcggcaagcccagacggaagaatcctcaagagggcctgtataatgagctgcagaaagacaagatggccgaggcctacagcgagatcggaatgaagggcgagcgcagaagaggcaagggacacgatggactgtaccagggcctgagcaccgccaccaaggatacctatgatgccctgcacatgcaggccctgcctccaagataa

SEQ ID NO: 70 - RNA, 2910 nt, Synthetic construct
  source 1..2910: mol_type = other RNA
atggctctgcctgttacagctctgctgctgcctctggctctgcttctgcatgccgctagacctgaggtgcagctggttgaatctggcgccgaagtgaagaaaccaggcgcctctgtgaaggtgtcctgcaaggtgtccggctacaccctgacagagctgagcatgcactgggtccgacaggcccctggaaaaggccttgaatggatgggcggcttcgaccccgaagatggcgagactatgtacgcccagaaattccagggcagagtgaccatgaccgaggacaccagcaccgacaccgcctacatggaactgagcagcctgagaagcgaggataccgccgtgtactactgcgccacatctacagccgtggccggcacacctgacctgttcgattactactacggcatggacgtgtggggccagggcacaacagtgacagtttcttctggcggcggaggatctggcggaggtggaagcggaggcggtggatctgagatcgtgatgacacagagccctctgtctagccccgtgacactgggacagcctgccagcatcagctgtagaagcagccagagcctggtgcacagcgacggcaatacctacctgtcttggctgcagcagaggcctggacagcctcctagactgctgatctacaagatcagcaaccggttcagcggcgtgcccgatagattttctggtagcggagccggcaccgacttcaccctgaagatcagtagagtggaagccgaggacgtgggcgtgtactattgcacacaggccacacagttcccttacaccttcggacagggcaccaaggtggacatcaaggactacaaggacgacgacgacaagcagctttcattaccctctatccttccaaatgaaaatgaaaaggttgtgcagctgaattcatccttttctctgagatgctttggggagagtgaagtgagctggcagtaccccatgtctgaagaagagagctccgatgtggaaatcagaaatgaagaaaacaacagcggcctttttgtgacggtcttggaagtgagcagtgcctcggcggcccacacagggttgtacacttgctattacaaccacactcagacagaagagaatgagcttgaaggcaggcacatttacatctatgtgccagacccagatgtagcctttgtacctctaggaatgacggattatttagtcatcgtggaggatgatgattctgccattataccttgtcgcacaactgatcccgagactcctgtaaccttacacaacagtgagggggtggtacctgcctcctacgacagcagacagggctttaatgggaccttcactgtagggccctatatctgtgaggccaccgtcaaaggaaagaagttccagaccatcccatttaatgtttatgctttaaaagcaacatcagagctggatctagaaatggaagctcttaaaaccgtgtataagtcaggggaaacgattgtggtcacctgtgctgtttttaacaatgaggtggttgaccttcaatggacttaccctggagaagtgaaaggcaaaggcatcacaatgctggaagaaatcaaagtcccatccatcaaattggtgtacactttgacggtccccgaggccacggtgaaagacagtggagattacgaatgtgctgcccgccaggctaccagggaggtcaaagaaatgaagaaagtcactatttctgtccatgagaaaggtttcattgaaatcaaacccaccttcagccagttggaagctgtcaacctgcatgaagtcaaacattttgttgtagaggtgcgggcctacccacctcccaggatatcctggctgaaaaacaatctgactctgattgaaaatctcactgagatcaccactgatgtggaaaagattcaggaaataaggtatcgaagcaaattaaagctgatccgtgctaaggaagaagacagtggccattatactattgtagctcaaaatgaagatgctgtgaagagctatacttttgaactgttaactcaagttccttcatccattctggacttggtcgatgatcaccatggctcaactgggggacagacggtgaggtgcacagctgaaggcacgccgcttcctgatattgagtggatgatatgcaaagatattaagaaatgtaataatgaaacttcctggactattttggccaacaatgtctcaaacatcatcacggagatccactcccgagacaggagtaccgtggagggccgtgtgactttcgccaaagtggaggagaccatcgccgtgcgatgcctggctaagaatctccttggagctgagaaccgagagctgaagctggtggctcccaccctgcgttctgaactcacggtggctttctgggtgctcgttgttgttggcggcgtgctggcctgttactctctgctggttaccgtggccttcatcatcttttgggtccgaagcaagcggagcagaggcggccacagcgactacatgaacatgacccctagacggcccggaccaaccagaaagcactaccagccttacgctcctcctagagacttcgccgcctaccggtccagagtgaagttcagcagatccgccgatgctcccgcctatcagcagggacagaaccagctgtacaacgagctgaacctggggagaagagaagagtacgacgtgctggacaagcggagaggcagagatcctgagatgggcggcaagcccagacggaagaatcctcaagagggcctgtataatgagctgcagaaagacaagatggccgaggcctacagcgagatcggaatgaagggcgagcgcagaagaggcaagggacacgatggactgtaccagggcctgagcaccgccaccaaggatacctatgatgccctgcacatgcaggccctgcctccaagataa

SEQ ID NO: 71 - DNA, 2895 bp, Synthetic construct
  source 1..2895: mol_type = other DNA
atggctctgcctgttacagctctgctgctgcctctggctctgcttctgcatgccgctagacctgaggtgcagctggttgaatctggcgccgaagtgaagaaaccaggcgcctctgtgaaggtgtcctgcaaggtgtccggctacaccctgacagagctgagcatgcactgggtccgacaggcccctggaaaaggccttgaatggatgggcggcttcgaccccgaagatggcgagactatgtacgcccagaaattccagggcagagtgaccatgaccgaggacaccagcaccgacaccgcctacatggaactgagcagcctgagaagcgaggataccgccgtgtactactgcgccacatctacagccgtggccggcacacctgacctgttcgattactactacggcatggacgtgtggggccagggcacaacagtgacagtttcttctggcggcggaggatctggcggaggtggaagcggaggcggtggatctgagatcgtgatgacacagagccctctgtctagccccgtgacactgggacagcctgccagcatcagctgtagaagcagccagagcctggtgcacagcgacggcaatacctacctgtcttggctgcagcagaggcctggacagcctcctagactgctgatctacaagatcagcaaccggttcagcggcgtgcccgatagattttctggtagcggagccggcaccgacttcaccctgaagatcagtagagtggaagccgaggacgtgggcgtgtactattgcacacaggccacacagttcccttacaccttcggacagggcaccaaggtggacatcaaggactacaaggacgacgacgacaagctggtcgtcacacccccggggccagagcttgtcctcaatgtctccagcaccttcgttctgacctgctcgggttcagctccggtggtgtgggaacggatgtcccaggagcccccacaggaaatggccaaggcccaggatggcaccttctccagcgtgctcacactgaccaacctcactgggctagacacgggagaatacttttgcacccacaatgactcccgtggactggagaccgatgagcggaaacggctctacatctttgtgccagatcccaccgtgggcttcctccctaatgatgccgaggaactattcatctttctcacggaaataactgagatcaccattccatgccgagtaacagacccacagctggtggtgacactgcacgagaagaaaggggacgttgcactgcctgtcccctatgatcaccaacgtggcttttttggtatctttgaggacagaagctacatctgcaaaaccaccattggggacagggaggtggattctgatgcctactatgtctacagactccaggtgtcatccatcaacgtctctgtgaacgcagtgcagactgtggtccgccagggtgagaacatcaccctcatgtgcattgtgatcgggaatgaggtggtcaacttcgagtggacatacccccgcaaagaaagtgggcggctggtggagccggtgactgacttcctcttggatatgccttaccacatccgctccatcctgcacatccccagtgccgagttagaagactcggggacctacacctgcaatgtgacggagagtgtgaatgaccatcaggatgaaaaggccatcaacatcaccgtggttgagagcggctacgtgcggctcctgggagaggtgggcacactacaatttgctgagctgcatcggagccggacactgcaggtagtgttcgaggcctacccaccgcccactgtcctgtggttcaaagacaaccgcaccctgggcgactccagcgctggcgaaatcgccctgtccacgcgcaacgtgtcggagacccggtatgtgtcagagctgacactggttcgcgtgaaggtggcagaggctggccactacaccatgcgggccttccatgaggatgctgaggtccagctctccttccagctacagatcaatgtccctgtccgagtgctggagctaagtgagagccaccctgacagtggggaacagacagtccgctgtcgtggccggggcatgccccagccgaacatcatctggtctgcctgcagagacctcaaaaggtgtccacgtgagctgccgcccacgctgctggggaacagttccgaagaggagagccagctggagactaacgtgacgtactgggaggaggagcaggagtttgaggtggtgagcacactgcgtctgcagcacgtggatcggccactgtcggtgcgctgcacgctgcgcaacgctgtgggccaggacacgcaggaggtcatcgtggtgccacactccttgccctttaaggtgttctgggtgctcgttgttgttggcggcgtgctggcctgttactctctgctggttaccgtggccttcatcatcttttgggtccgaagcaagcggagcagaggcggccacagcgactacatgaacatgacccctagacggcccggaccaaccagaaagcactaccagccttacgctcctcctagagacttcgccgcctaccggtccagagtgaagttcagcagatccgccgatgctcccgcctatcagcagggacagaaccagctgtacaacgagctgaacctggggagaagagaagagtacgacgtgctggacaagcggagaggcagagatcctgagatgggcggcaagcccagacggaagaatcctcaagagggcctgtataatgagctgcagaaagacaagatggccgaggcctacagcgagatcggaatgaagggcgagcgcagaagaggcaagggacacgatggactgtaccagggcctgagcaccgccaccaaggatacctatgatgccctgcacatgcaggccctgcctccaagataa

SEQ ID NO: 72 - RNA, 2895 nt, Synthetic construct
  source 1..2895: mol_type = other RNA
atggctctgcctgttacagctctgctgctgcctctggctctgcttctgcatgccgctagacctgaggtgcagctggttgaatctggcgccgaagtgaagaaaccaggcgcctctgtgaaggtgtcctgcaaggtgtccggctacaccctgacagagctgagcatgcactgggtccgacaggcccctggaaaaggccttgaatggatgggcggcttcgaccccgaagatggcgagactatgtacgcccagaaattccagggcagagtgaccatgaccgaggacaccagcaccgacaccgcctacatggaactgagcagcctgagaagcgaggataccgccgtgtactactgcgccacatctacagccgtggccggcacacctgacctgttcgattactactacggcatggacgtgtggggccagggcacaacagtgacagtttcttctggcggcggaggatctggcggaggtggaagcggaggcggtggatctgagatcgtgatgacacagagccctctgtctagccccgtgacactgggacagcctgccagcatcagctgtagaagcagccagagcctggtgcacagcgacggcaatacctacctgtcttggctgcagcagaggcctggacagcctcctagactgctgatctacaagatcagcaaccggttcagcggcgtgcccgatagattttctggtagcggagccggcaccgacttcaccctgaagatcagtagagtggaagccgaggacgtgggcgtgtactattgcacacaggccacacagttcccttacaccttcggacagggcaccaaggtggacatcaaggactacaaggacgacgacgacaagctggtcgtcacacccccggggccagagcttgtcctcaatgtctccagcaccttcgttctgacctgctcgggttcagctccggtggtgtgggaacggatgtcccaggagcccccacaggaaatggccaaggcccaggatggcaccttctccagcgtgctcacactgaccaacctcactgggctagacacgggagaatacttttgcacccacaatgactcccgtggactggagaccgatgagcggaaacggctctacatctttgtgccagatcccaccgtgggcttcctccctaatgatgccgaggaactattcatctttctcacggaaataactgagatcaccattccatgccgagtaacagacccacagctggtggtgacactgcacgagaagaaaggggacgttgcactgcctgtcccctatgatcaccaacgtggcttttttggtatctttgaggacagaagctacatctgcaaaaccaccattggggacagggaggtggattctgatgcctactatgtctacagactccaggtgtcatccatcaacgtctctgtgaacgcagtgcagactgtggtccgccagggtgagaacatcaccctcatgtgcattgtgatcgggaatgaggtggtcaacttcgagtggacatacccccgcaaagaaagtgggcggctggtggagccggtgactgacttcctcttggatatgccttaccacatccgctccatcctgcacatccccagtgccgagttagaagactcggggacctacacctgcaatgtgacggagagtgtgaatgaccatcaggatgaaaaggccatcaacatcaccgtggttgagagcggctacgtgcggctcctgggagaggtgggcacactacaatttgctgagctgcatcggagccggacactgcaggtagtgttcgaggcctacccaccgcccactgtcctgtggttcaaagacaaccgcaccctgggcgactccagcgctggcgaaatcgccctgtccacgcgcaacgtgtcggagacccggtatgtgtcagagctgacactggttcgcgtgaaggtggcagaggctggccactacaccatgcgggccttccatgaggatgctgaggtccagctctccttccagctacagatcaatgtccctgtccgagtgctggagctaagtgagagccaccctgacagtggggaacagacagtccgctgtcgtggccggggcatgccccagccgaacatcatctggtctgcctgcagagacctcaaaaggtgtccacgtgagctgccgcccacgctgctggggaacagttccgaagaggagagccagctggagactaacgtgacgtactgggaggaggagcaggagtttgaggtggtgagcacactgcgtctgcagcacgtggatcggccactgtcggtgcgctgcacgctgcgcaacgctgtgggccaggacacgcaggaggtcatcgtggtgccacactccttgccctttaaggtgttctgggtgctcgttgttgttggcggcgtgctggcctgttactctctgctggttaccgtggccttcatcatcttttgggtccgaagcaagcggagcagaggcggccacagcgactacatgaacatgacccctagacggcccggaccaaccagaaagcactaccagccttacgctcctcctagagacttcgccgcctaccggtccagagtgaagttcagcagatccgccgatgctcccgcctatcagcagggacagaaccagctgtacaacgagctgaacctggggagaagagaagagtacgacgtgctggacaagcggagaggcagagatcctgagatgggcggcaagcccagacggaagaatcctcaagagggcctgtataatgagctgcagaaagacaagatggccgaggcctacagcgagatcggaatgaagggcgagcgcagaagaggcaagggacacgatggactgtaccagggcctgagcaccgccaccaaggatacctatgatgccctgcacatgcaggccctgcctccaagataa

SEQ ID NO: 73 - DNA, 1827 bp, Synthetic construct
  source 1..1827: mol_type = other DNA
atggctctgcctgttacagctctgctgctgcctctggctctgcttctgcatgccgctagacctgaggtgcagctggttgaatctggcgccgaagtgaagaaaccaggcgcctctgtgaaggtgtcctgcaaggtgtccggctacaccctgacagagctgagcatgcactgggtccgacaggcccctggaaaaggccttgaatggatgggcggcttcgaccccgaagatggcgagactatgtacgcccagaaattccagggcagagtgaccatgaccgaggacaccagcaccgacaccgcctacatggaactgagcagcctgagaagcgaggataccgccgtgtactactgcgccacatctacagccgtggccggcacacctgacctgttcgattactactacggcatggacgtgtggggccagggcacaacagtgacagtttcttctggcggcggaggatctggcggaggtggaagcggaggcggtggatctgagatcgtgatgacacagagccctctgtctagccccgtgacactgggacagcctgccagcatcagctgtagaagcagccagagcctggtgcacagcgacggcaatacctacctgtcttggctgcagcagaggcctggacagcctcctagactgctgatctacaagatcagcaaccggttcagcggcgtgcccgatagattttctggtagcggagccggcaccgacttcaccctgaagatcagtagagtggaagccgaggacgtgggcgtgtactattgcacacaggccacacagttcccttacaccttcggacagggcaccaaggtggacatcaaggactacaaggacgacgacgacaagcaagaagaggacctgcctagacctagcatctctgccgagcctggcacagtgatccctctgggaagccacgtgaccttcgtgtgtagaggaccagtgggcgtgcagaccttccggctggaaagagagagcagaagcacctacaacgacaccgaggacgtgtcccaggcctctccatctgagagcgaggccagattcagaatcgacagcgtgtccgagggcaacgctggcccttaccggtgcatctactacaagcctccaaagtggagcgagcagagcgactacctggaactgctggtcaaagagacatctggcggccctgacagccctgatacagagcctggatctagcgccggacctacacagaggcccagcgacaatagccacaatgaacacgcccctgccagccagggactgaaagccgaacatctgtacttctgggtgctcgttgttgttggcggcgtgctggcctgttactctctgctggttaccgtggccttcatcatcttttgggtccgaagcaagcggagcagaggcggccacagcgactacatgaacatgacccctagacggcccggaccaaccagaaagcactaccagccttacgctcctcctagagacttcgccgcctaccggtccagagtgaagttcagcagatccgccgatgctcccgcctatcagcagggacagaaccagctgtacaacgagctgaacctggggagaagagaagagtacgacgtgctggacaagcggagaggcagagatcctgagatgggcggcaagcccagacggaagaatcctcaagagggcctgtataatgagctgcagaaagacaagatggccgaggcctacagcgagatcggaatgaagggcgagcgcagaagaggcaagggacacgatggactgtaccagggcctgagcaccgccaccaaggatacctatgatgccctgcacatgcaggccctgcctccaagataa

SEQ ID NO: 74 - RNA, 1827 nt, Synthetic construct
  source 1..1827: mol_type = other RNA
atggctctgcctgttacagctctgctgctgcctctggctctgcttctgcatgccgctagacctgaggtgcagctggttgaatctggcgccgaagtgaagaaaccaggcgcctctgtgaaggtgtcctgcaaggtgtccggctacaccctgacagagctgagcatgcactgggtccgacaggcccctggaaaaggccttgaatggatgggcggcttcgaccccgaagatggcgagactatgtacgcccagaaattccagggcagagtgaccatgaccgaggacaccagcaccgacaccgcctacatggaactgagcagcctgagaagcgaggataccgccgtgtactactgcgccacatctacagccgtggccggcacacctgacctgttcgattactactacggcatggacgtgtggggccagggcacaacagtgacagtttcttctggcggcggaggatctggcggaggtggaagcggaggcggtggatctgagatcgtgatgacacagagccctctgtctagccccgtgacactgggacagcctgccagcatcagctgtagaagcagccagagcctggtgcacagcgacggcaatacctacctgtcttggctgcagcagaggcctggacagcctcctagactgctgatctacaagatcagcaaccggttcagcggcgtgcccgatagattttctggtagcggagccggcaccgacttcaccctgaagatcagtagagtggaagccgaggacgtgggcgtgtactattgcacacaggccacacagttcccttacaccttcggacagggcaccaaggtggacatcaaggactacaaggacgacgacgacaagcaagaagaggacctgcctagacctagcatctctgccgagcctggcacagtgatccctctgggaagccacgtgaccttcgtgtgtagaggaccagtgggcgtgcagaccttccggctggaaagagagagcagaagcacctacaacgacaccgaggacgtgtcccaggcctctccatctgagagcgaggccagattcagaatcgacagcgtgtccgagggcaacgctggcccttaccggtgcatctactacaagcctccaaagtggagcgagcagagcgactacctggaactgctggtcaaagagacatctggcggccctgacagccctgatacagagcctggatctagcgccggacctacacagaggcccagcgacaatagccacaatgaacacgcccctgccagccagggactgaaagccgaacatctgtacttctgggtgctcgttgttgttggcggcgtgctggcctgttactctctgctggttaccgtggccttcatcatcttttgggtccgaagcaagcggagcagaggcggccacagcgactacatgaacatgacccctagacggcccggaccaaccagaaagcactaccagccttacgctcctcctagagacttcgccgcctaccggtccagagtgaagttcagcagatccgccgatgctcccgcctatcagcagggacagaaccagctgtacaacgagctgaacctggggagaagagaagagtacgacgtgctggacaagcggagaggcagagatcctgagatgggcggcaagcccagacggaagaatcctcaagagggcctgtataatgagctgcagaaagacaagatggccgaggcctacagcgagatcggaatgaagggcgagcgcagaagaggcaagggacacgatggactgtaccagggcctgagcaccgccaccaaggatacctatgatgccctgcacatgcaggccctgcctccaagataa

SEQ ID NO: 75 - DNA, 1539 bp, Synthetic construct
  source 1..1539: mol_type = other DNA
atggctctgcctgttacagctctgctgctgcctctggctctgcttctgcatgccgctagacctgaggtgcagctggttgaatctggcgccgaagtgaagaaaccaggcgcctctgtgaaggtgtcctgcaaggtgtccggctacaccctgacagagctgagcatgcactgggtccgacaggcccctggaaaaggccttgaatggatgggcggcttcgaccccgaagatggcgagactatgtacgcccagaaattccagggcagagtgaccatgaccgaggacaccagcaccgacaccgcctacatggaactgagcagcctgagaagcgaggataccgccgtgtactactgcgccacatctacagccgtggccggcacacctgacctgttcgattactactacggcatggacgtgtggggccagggcacaacagtgacagtttcttctggcggcggaggatctggcggaggtggaagcggaggcggtggatctgagatcgtgatgacacagagccctctgtctagccccgtgacactgggacagcctgccagcatcagctgtagaagcagccagagcctggtgcacagcgacggcaatacctacctgtcttggctgcagcagaggcctggacagcctcctagactgctgatctacaagatcagcaaccggttcagcggcgtgcccgatagattttctggtagcggagccggcaccgacttcaccctgaagatcagtagagtggaagccgaggacgtgggcgtgtactattgcacacaggccacacagttcccttacaccttcggacagggcaccaaggtggacatcaaggactacaaggacgacgacgacaagctgctggtcaaagagacatctggcggccctgacagccctgatacagagcctggatctagcgccggacctacacagaggcccagcgacaatagccacaatgaacacgcccctgccagccagggactgaaagccgaacatctgtacttctgggtgctcgttgttgttggcggcgtgctggcctgttactctctgctggttaccgtggccttcatcatcttttgggtccgaagcaagcggagcagaggcggccacagcgactacatgaacatgacccctagacggcccggaccaaccagaaagcactaccagccttacgctcctcctagagacttcgccgcctaccggtccagagtgaagttcagcagatccgccgatgctcccgcctatcagcagggacagaaccagctgtacaacgagctgaacctggggagaagagaagagtacgacgtgctggacaagcggagaggcagagatcctgagatgggcggcaagcccagacggaagaatcctcaagagggcctgtataatgagctgcagaaagacaagatggccgaggcctacagcgagatcggaatgaagggcgagcgcagaagaggcaagggacacgatggactgtaccagggcctgagcaccgccaccaaggatacctatgatgccctgcacatgcaggccctgcctccaagataa

SEQ ID NO: 76 - RNA, 1539 nt, Synthetic construct
  source 1..1539: mol_type = other RNA
atggctctgcctgttacagctctgctgctgcctctggctctgcttctgcatgccgctagacctgaggtgcagctggttgaatctggcgccgaagtgaagaaaccaggcgcctctgtgaaggtgtcctgcaaggtgtccggctacaccctgacagagctgagcatgcactgggtccgacaggcccctggaaaaggccttgaatggatgggcggcttcgaccccgaagatggcgagactatgtacgcccagaaattccagggcagagtgaccatgaccgaggacaccagcaccgacaccgcctacatggaactgagcagcctgagaagcgaggataccgccgtgtactactgcgccacatctacagccgtggccggcacacctgacctgttcgattactactacggcatggacgtgtggggccagggcacaacagtgacagtttcttctggcggcggaggatctggcggaggtggaagcggaggcggtggatctgagatcgtgatgacacagagccctctgtctagccccgtgacactgggacagcctgccagcatcagctgtagaagcagccagagcctggtgcacagcgacggcaatacctacctgtcttggctgcagcagaggcctggacagcctcctagactgctgatctacaagatcagcaaccggttcagcggcgtgcccgatagattttctggtagcggagccggcaccgacttcaccctgaagatcagtagagtggaagccgaggacgtgggcgtgtactattgcacacaggccacacagttcccttacaccttcggacagggcaccaaggtggacatcaaggactacaaggacgacgacgacaagctgctggtcaaagagacatctggcggccctgacagccctgatacagagcctggatctagcgccggacctacacagaggcccagcgacaatagccacaatgaacacgcccctgccagccagggactgaaagccgaacatctgtacttctgggtgctcgttgttgttggcggcgtgctggcctgttactctctgctggttaccgtggccttcatcatcttttgggtccgaagcaagcggagcagaggcggccacagcgactacatgaacatgacccctagacggcccggaccaaccagaaagcactaccagccttacgctcctcctagagacttcgccgcctaccggtccagagtgaagttcagcagatccgccgatgctcccgcctatcagcagggacagaaccagctgtacaacgagctgaacctggggagaagagaagagtacgacgtgctggacaagcggagaggcagagatcctgagatgggcggcaagcccagacggaagaatcctcaagagggcctgtataatgagctgcagaaagacaagatggccgaggcctacagcgagatcggaatgaagggcgagcgcagaagaggcaagggacacgatggactgtaccagggcctgagcaccgccaccaaggatacctatgatgccctgcacatgcaggccctgcctccaagataa

SEQ ID NO: 77 - DNA, 2040 bp, Synthetic construct
  source 1..2040: mol_type = other DNA
atggctctgcctgtgacagctctgctgctgcctctggctctgcttctgcatgccgccagacctgacatccagatgacacagagccctagcagcctgtctgccagcgtgggagacagagtgaccatcacctgtagagccagccagagcatcagctcctacctgaactggtatcagcagaagcccggcaaggcccctaagctgctgatctatgctgccagctctctgcagtctggcgtgcccagcagattttctggcagcggctctggcaccgacttcaccctgaccatatctagcctgcagcctgaggacttcgccacctactactgccagcagtcctacagcacccctcctacatttggccagggcaccaaggtggaaatcaaaggcggcggaggatctggcggaggtggaagtggcggaggcggatctgaagtgcagctggttgaatcaggtggcggcctggttcaacctggcggatctctgagactgagctgtgccgccagcggcttcaccttcagcgaccactatatggactgggtccgacaggcccctggcaaaggacttgagtgggtcggacggaccagaaacaaggccaacagctacaccacagagtacgccgcctctgtgaagggcagattcaccatcagccgggacgacagcaagaacagcctgtacctgcagatgaactccctgaaaaccgaggacaccgccgtgtactactgcgccagaggaatcagccccttctacttcgactattggggccagggaaccctcgtgaccgtttcttctgactacaaggacgacgacgacaaggaatctaagtacggccctccttgtcctccatgtcctgctccacctgtggccggaccctccgtgttcctgtttcctccaaagcctaaggacaccctgatgatcagcagaacccctgaagtgacctgcgtggtggtggacgtttcccaagaggaccctgaggtgcagttcaattggtacgtggacggcgtggaagtgcacaacgccaagaccaagcctagagaggaacagttccagagcacctacagagtggtgtccgtgctgaccgtgctgcaccaggattggctgaacggcaaagagtacaagtgcaaggtgtccaacaagggcctgcctagcagcatcgagaaaaccatcagcaaggccaagggccagccaagagaaccccaggtgtacacactgcctccaagccaagaggaaatgaccaagaaccaggtgtccctgacctgcctggtcaagggcttctacccttccgatatcgccgtggaatgggagagcaatggccagcctgagaacaactacaagaccacacctcctgtgctggacagcgacggctcattcttcctgtacagcagactgaccgtggacaagagcagatggcaagagggcaacgtgttcagctgcagcgtgatgcacgaggccctgcacaaccactacacccagaagtctctgagcctgagcctgggcaagttctgggtgctcgttgttgttggcggcgtgctggcctgttactctctgctggttaccgtggccttcatcatcttttgggtccgaagcaagcggagcagaggcggccacagcgactacatgaacatgacccctagacggcccggaccaaccagaaagcactaccagccttacgctcctcctagagacttcgccgcctaccggtccagagtgaagttcagcagatccgccgatgctcccgcctatcagcagggacagaaccagctgtacaacgagctgaacctggggagaagagaagagtacgacgtgctggacaagcggagaggcagagatcctgagatgggcggcaagcccagacggaagaatcctcaagagggcctgtataatgagctgcagaaagacaagatggccgaggcctacagcgagatcggaatgaagggcgagcgcagaagaggcaagggacacgatggactgtaccagggcctgagcaccgccaccaaggatacctatgatgccctgcacatgcaggccctgcctccaagataa

SEQ ID NO: 78 - RNA, 2040 nt, Synthetic construct
  source 1..2040: mol_type = other RNA
atggctctgcctgtgacagctctgctgctgcctctggctctgcttctgcatgccgccagacctgacatccagatgacacagagccctagcagcctgtctgccagcgtgggagacagagtgaccatcacctgtagagccagccagagcatcagctcctacctgaactggtatcagcagaagcccggcaaggcccctaagctgctgatctatgctgccagctctctgcagtctggcgtgcccagcagattttctggcagcggctctggcaccgacttcaccctgaccatatctagcctgcagcctgaggacttcgccacctactactgccagcagtcctacagcacccctcctacatttggccagggcaccaaggtggaaatcaaaggcggcggaggatctggcggaggtggaagtggcggaggcggatctgaagtgcagctggttgaatcaggtggcggcctggttcaacctggcggatctctgagactgagctgtgccgccagcggcttcaccttcagcgaccactatatggactgggtccgacaggcccctggcaaaggacttgagtgggtcggacggaccagaaacaaggccaacagctacaccacagagtacgccgcctctgtgaagggcagattcaccatcagccgggacgacagcaagaacagcctgtacctgcagatgaactccctgaaaaccgaggacaccgccgtgtactactgcgccagaggaatcagccccttctacttcgactattggggccagggaaccctcgtgaccgtttcttctgactacaaggacgacgacgacaaggaatctaagtacggccctccttgtcctccatgtcctgctccacctgtggccggaccctccgtgttcctgtttcctccaaagcctaaggacaccctgatgatcagcagaacccctgaagtgacctgcgtggtggtggacgtttcccaagaggaccctgaggtgcagttcaattggtacgtggacggcgtggaagtgcacaacgccaagaccaagcctagagaggaacagttccagagcacctacagagtggtgtccgtgctgaccgtgctgcaccaggattggctgaacggcaaagagtacaagtgcaaggtgtccaacaagggcctgcctagcagcatcgagaaaaccatcagcaaggccaagggccagccaagagaaccccaggtgtacacactgcctccaagccaagaggaaatgaccaagaaccaggtgtccctgacctgcctggtcaagggcttctacccttccgatatcgccgtggaatgggagagcaatggccagcctgagaacaactacaagaccacacctcctgtgctggacagcgacggctcattcttcctgtacagcagactgaccgtggacaagagcagatggcaagagggcaacgtgttcagctgcagcgtgatgcacgaggccctgcacaaccactacacccagaagtctctgagcctgagcctgggcaagttctgggtgctcgttgttgttggcggcgtgctggcctgttactctctgctggttaccgtggccttcatcatcttttgggtccgaagcaagcggagcagaggcggccacagcgactacatgaacatgacccctagacggcccggaccaaccagaaagcactaccagccttacgctcctcctagagacttcgccgcctaccggtccagagtgaagttcagcagatccgccgatgctcccgcctatcagcagggacagaaccagctgtacaacgagctgaacctggggagaagagaagagtacgacgtgctggacaagcggagaggcagagatcctgagatgggcggcaagcccagacggaagaatcctcaagagggcctgtataatgagctgcagaaagacaagatggccgaggcctacagcgagatcggaatgaagggcgagcgcagaagaggcaagggacacgatggactgtaccagggcctgagcaccgccaccaaggatacctatgatgccctgcacatgcaggccctgcctccaagataa

SEQ ID NO: 79 - protein, 1270 aa, Synthetic construct
MFVFLVLLPLVSSQCVNLTTRTQLPPAYTNSFTRGVYYPDKVFRSSVLHSTQDLFLPFFSNVTWFHVISGTNGTKRFDNPVLPFNDGVYFASIEKSNIIRGWIFGTTLDSKTQSLLIVNNATNVVIKVCEFQFCNDPFLDHKNNKSWMESEFRVYSSANNCTFEYVSQPFLMDLEGKQGNFKNLREFVFKNIDGYFKIYSKHTPIIVREPEDLPQGFSALEPLVDLPIGINITRFQTLLALHRSYLTPGDSSSGWTAGAAAYYVGYLQPRTFLLKYNENGTITDAVDCALDPLSETKCTLKSFTVEKGIYQTSNFRVQPTESIVRFPNITNLCPFDEVFNATRFASVYAWNRKRISNCVADYSVLYNLAPFFTFKCYGVSPTKLNDLCFTNVYADSFVIRGDEVRQIAPGQTGNIADYNYKLPDDFTGCVIAWNSNKLDSKVSGNYNYLYRLFRKSNLKPFERDISTEIYQAGNKPCNGVAGFNCYFPLRSYSFRPTYGVGHQPYRVVVLSFELLHAPATVCGPKKSTNLVKNKCVNFNFNGLKGTGVLTESNKKFLPFQQFGRDIADTTDAVRDPQTLEILDITPCSFGGVSVITPGTNTSNQVAVLYQGVNCTEVPVAIHADQLTPTWRVYSTGSNVFQTRAGCLIGAEYVNNSYECDIPIGAGICASYQTQTKSHRRARSVASQSIIAYTMSLGAENSVAYSNNSIAIPTNFTISVTTEILPVSMTKTSVDCTMYICGDSTECSNLLLQYGSFCTQLKRALTGIAVEQDKNTQEVFAQVKQIYKTPPIKYFGGFNFSQILPDPSKPSKRSFIEDLLFNKVTLADAGFIKQYGDCLGDIAARDLICAQKFKGLTVLPPLLTDEMIAQYTSALLAGTITSGWTFGAGAALQIPFAMQMAYRFNGIGVTQNVLYENQKLIANQFNSAIGKIQDSLSSTASALGKLQDVVNHNAQALNTLVKQLSSKFGAISSVLNDIFSRLDKVEAEVQIDRLITGRLQSLQTYVTQQLIRAAEIRASANLAATKMSECVLGQSKRVDFCGKGYHLMSFPQSAPHGVVFLHVTYVPAQEKNFTTAPAICHDGKAHFPREGVFVSNGTHWFVTQRNFYEPQIITTDNTFVSGNCDVVIGIVNNTVYDPLQPELDSFKEELDKYFKNHTSPDVDLGDISGINASVVNIQKEIDRLNEVAKNLNESLIDLQELGKYEQYIKWPWYIWLGFIAGLIAIVMVTIMLCCMTSCCSCLKGCCSCGSCCKFDEDDSEPVLKGVKLHYT

SEQ ID NO: 80 - protein, 248 aa, Synthetic construct
MALPVTALLLPLALLLHAARPDYKDDDDKIEVMYPPPYLDNEKSNGTIIHVKGKHLCPSPLFPGPSKPFWVLVVVGGVLACYSLLVTVAFIIFWVRSKRSRGGHSDYMNMTPRRPGPTRKHYQPYAPPRDFAAYRSRVKFSRSADAPAYQQGQNQLYNELNLGRREEYDVLDKRRGRDPEMGGKPRRKNPQEGLYNELQKDKMAEAYSEIGMKGERRRGKGHDGLYQGLSTATKDTYDALHMQALPPR

SEQ ID NO: 81 - protein, 490 aa, Synthetic construct
MALPVTALLLPLALLLHAARPDIQMTQSPSSLSASVGDRVTITCRASQSISSYLNWYQQKPGKAPKLLIYAASSLQSGVPSRFSGSGSGTDFTLTISSLQPEDFATYYCQQSYSTPPTFGQGTKVEIKGGGGSGGGGSGGGGSEVQLVESGGGLVQPGGSLRLSCAASGFTFSDHYMDWVRQAPGKGLEWVGRTRNKANSYTTEYAASVKGRFTISRDDSKNSLYLQMNSLKTEDTAVYYCARGISPFYFDYWGQGTLVTVSSDYKDDDDKIEVMYPPPYLDNEKSNGTIIHVKGKHLCPSPLFPGPSKPFWVLVVVGGVLACYSLLVTVAFIIFWVRSKRSRGGHSDYMNMTPRRPGPTRKHYQPYAPPRDFAAYRSRVKFSRSADAPAYQQGQNQLYNELNLGRREEYDVLDKRRGRDPEMGGKPRRKNPQEGLYNELQKDKMAEAYSEIGMKGERRRGKGHDGLYQGLSTATKDTYDALHMQALPPR

SEQ ID NO: 82 - protein, 495 aa, Synthetic construct
MALPVTALLLPLALLLHAARPDIVMTQSPDSLAVSLGERATINCKSSQSVLYSSINKNYLAWYQQKPGQPPKLLIYWASTRESGVPDRFSGSGSGTDFTLTISSLQAEDVAVYYCQQYYSTPYTFGQGTKVEIKGGGGSGGGGSGGGGSEVQLVQSGTEVKKPGESLKISCKGSGYGFITYWIGWVRQMPGKGLEWMGIIYPGDSETRYSPSFQGQVTISADKSINTAYLQWSSLKASDTAIYYCAGGSGISTPMDVWGQGTTVTVSSDYKDDDDKIEVMYPPPYLDNEKSNGTIIHVKGKHLCPSPLFPGPSKPFWVLVVVGGVLACYSLLVTVAFIIFWVRSKRSRGGHSDYMNMTPRRPGPTRKHYQPYAPPRDFAAYRSRVKFSRSADAPAYQQGQNQLYNELNLGRREEYDVLDKRRGRDPEMGGKPRRKNPQEGLYNELQKDKMAEAYSEIGMKGERRRGKGHDGLYQGLSTATKDTYDALHMQALPPR

SEQ ID NO: 83 - protein, 503 aa, Synthetic construct
MALPVTALLLPLALLLHAARPDIVMTQSPDSLAVSLGERATINCKSSQSVLYSSINKNYLAWYQQKPGQPPKLLIYWASTRESGVPDRFSGSGSGTDFTLTISSLQAEDVAVYYCQQYYSTPYTFGQGTKVEIKGGGGSGGGGSGGGGSEVQLVQSGTEVKKPGESLKISCKGSGYGFITYWIGWVRQMPGKGLEWMGIIYPGDSETRYSPSFQGQVTISADKSINTAYLQWSSLKASDTAIYYCAGGSGISTPMDVWGQGTTVTVSSDYKDDDDKKPTTTPAPRPPTPAPTIASQPLSLRPEACRPAAGGAVHTRGLDFACDFWVLVVVGGVLACYSLLVTVAFIIFWVRSKRSRGGHSDYMNMTPRRPGPTRKHYQPYAPPRDFAAYRSRVKFSRSADAPAYQQGQNQLYNELNLGRREEYDVLDKRRGRDPEMGGKPRRKNPQEGLYNELQKDKMAEAYSEIGMKGERRRGKGHDGLYQGLSTATKDTYDALHMQALPPR

SEQ ID NO: 84 - protein, 575 aa, Synthetic construct
MALPVTALLLPLALLLHAARPDIVMTQSPDSLAVSLGERATINCKSSQSVLYSSINKNYLAWYQQKPGQPPKLLIYWASTRESGVPDRFSGSGSGTDFTLTISSLQAEDVAVYYCQQYYSTPYTFGQGTKVEIKGGGGSGGGGSGGGGSEVQLVQSGTEVKKPGESLKISCKGSGYGFITYWIGWVRQMPGKGLEWMGIIYPGDSETRYSPSFQGQVTISADKSINTAYLQWSSLKASDTAIYYCAGGSGISTPMDVWGQGTTVTVSSDYKDDDDKESKYGPPCPPCPGQPREPQVYTLPPSQEEMTKNQVSLTCLVKGFYPSDIAVEWESNGQPENNYKTTPPVLDSDGSFFLYSRLTVDKSRWQEGNVFSCSVMHEALHNHYTQKSLSLSLGKFWVLVVVGGVLACYSLLVTVAFIIFWVRSKRSRGGHSDYMNMTPRRPGPTRKHYQPYAPPRDFAAYRSRVKFSRSADAPAYQQGQNQLYNELNLGRREEYDVLDKRRGRDPEMGGKPRRKNPQEGLYNELQKDKMAEAYSEIGMKGERRRGKGHDGLYQGLSTATKDTYDALHMQALPPR

SEQ ID NO: 85 - protein, 685 aa, Synthetic construct
MALPVTALLLPLALLLHAARPDIVMTQSPDSLAVSLGERATINCKSSQSVLYSSINKNYLAWYQQKPGQPPKLLIYWASTRESGVPDRFSGSGSGTDFTLTISSLQAEDVAVYYCQQYYSTPYTFGQGTKVEIKGGGGSGGGGSGGGGSEVQLVQSGTEVKKPGESLKISCKGSGYGFITYWIGWVRQMPGKGLEWMGIIYPGDSETRYSPSFQGQVTISADKSINTAYLQWSSLKASDTAIYYCAGGSGISTPMDVWGQGTTVTVSSDYKDDDDKESKYGPPCPPCPAPEFLGGPSVFLFPPKPKDTLMISRTPEVTCVVVDVSQEDPEVQFNWYVDGVEVHNAKTKPREEQFNSTYRVVSVLTVLHQDWLNGKEYKCKVSNKGLPSSIEKTISKAKGQPREPQVYTLPPSQEEMTKNQVSLTCLVKGFYPSDIAVEWESNGQPENNYKTTPPVLDSDGSFFLYSRLTVDKSRWQEGNVFSCSVMHEALHNHYTQKSLSLSLGKFWVLVVVGGVLACYSLLVTVAFIIFWVRSKRSRGGHSDYMNMTPRRPGPTRKHYQPYAPPRDFAAYRSRVKFSRSADAPAYQQGQNQLYNELNLGRREEYDVLDKRRGRDPEMGGKPRRKNPQEGLYNELQKDKMAEAYSEIGMKGERRRGKGHDGLYQGLSTATKDTYDALHMQALPPR

SEQ ID NO: 86 - protein, 678 aa, Synthetic construct
MALPVTALLLPLALLLHAARPQVQLVESGGGVVQPGRSLRLSCAASGFTFSSYAMHWVRQAPGKGLEWVAVIPFDGRNKYYADSVTGRFTISRDNSKNTLYLQMNSLRAEDTAVYYCASSSGYLFHSDYWGQGTLVTVSSGGGGSGGGGSGGGGSDIQMTQSPSTLSASVGDRVTITCRASQSISNWLAWFQQKPGKAPKLLIYEASSLESGVPSRFSGSGSGTEFTLTISSLQPDDFATYYCQQYNSYPWTFGQGTKVEIKDYKDDDDKESKYGPPCPPCPAPPVAGPSVFLFPPKPKDTLMISRTPEVTCVVVDVSQEDPEVQFNWYVDGVEVHNAKTKPREEQFQSTYRVVSVLTVLHQDWLNGKEYKCKVSNKGLPSSIEKTISKAKGQPREPQVYTLPPSQEEMTKNQVSLTCLVKGFYPSDIAVEWESNGQPENNYKTTPPVLDSDGSFFLYSRLTVDKSRWQEGNVFSCSVMHEALHNHYTQKSLSLSLGKFWVLVVVGGVLACYSLLVTVAFIIFWVRSKRSRGGHSDYMNMTPRRPGPTRKHYQPYAPPRDFAAYRSRVKFSRSADAPAYQQGQNQLYNELNLGRREEYDVLDKRRGRDPEMGGKPRRKNPQEGLYNELQKDKMAEAYSEIGMKGERRRGKGHDGLYQGLSTATKDTYDALHMQALPPR

SEQ ID NO: 87 - protein, 686 aa, Synthetic construct
MALPVTALLLPLALLLHAARPQVQLVQSGAEVKKPGASVKVSCKASGYPFTSYGISWVRQAPGQGLEWMGWISTYNGNTNYAQKFQGRVTMTTDTSTTTGYMELRRLRSDDTAVYYCARDYTRGAWFGESLIGGFDNWGQGTLVTVSSGGGGSGGGGSGGGGSEIVLTQSPGTLSLSPGERATLSCRASQTVSSTSLAWYQQKPGQAPRLLIYGASSRATGIPDRFSGSGSGTDFTLTISRLEPEDFAVYYCQQHDTSLTFGGGTKVEIKDYKDDDDKESKYGPPCPPCPAPPVAGPSVFLFPPKPKDTLMISRTPEVTCVVVDVSQEDPEVQFNWYVDGVEVHNAKTKPREEQFQSTYRVVSVLTVLHQDWLNGKEYKCKVSNKGLPSSIEKTISKAKGQPREPQVYTLPPSQEEMTKNQVSLTCLVKGFYPSDIAVEWESNGQPENNYKTTPPVLDSDGSFFLYSRLTVDKSRWQEGNVFSCSVMHEALHNHYTQKSLSLSLGKFWVLVVVGGVLACYSLLVTVAFIIFWVRSKRSRGGHSDYMNMTPRRPGPTRKHYQPYAPPRDFAAYRSRVKFSRSADAPAYQQGQNQLYNELNLGRREEYDVLDKRRGRDPEMGGKPRRKNPQEGLYNELQKDKMAEAYSEIGMKGERRRGKGHDGLYQGLSTATKDTYDALHMQALPPR

SEQ ID NO: 88 - protein, 692 aa, Synthetic construct
MALPVTALLLPLALLLHAARPEVQLVESGAEVKKPGASVKVSCKVSGYTLTELSMHWVRQAPGKGLEWMGGFDPEDGETMYAQKFQGRVTMTEDTSTDTAYMELSSLRSEDTAVYYCATSTAVAGTPDLFDYYYGMDVWGQGTTVTVSSGGGGSGGGGSGGGGSEIVMTQSPLSSPVTLGQPASISCRSSQSLVHSDGNTYLSWLQQRPGQPPRLLIYKISNRFSGVPDRFSGSGAGTDFTLKISRVEAEDVGVYYCTQATQFPYTFGQGTKVDIKDYKDDDDKESKYGPPCPPCPAPPVAGPSVFLFPPKPKDTLMISRTPEVTCVVVDVSQEDPEVQFNWYVDGVEVHNAKTKPREEQFQSTYRVVSVLTVLHQDWLNGKEYKCKVSNKGLPSSIEKTISKAKGQPREPQVYTLPPSQEEMTKNQVSLTCLVKGFYPSDIAVEWESNGQPENNYKTTPPVLDSDGSFFLYSRLTVDKSRWQEGNVFSCSVMHEALHNHYTQKSLSLSLGKFWVLVVVGGVLACYSLLVTVAFIIFWVRSKRSRGGHSDYMNMTPRRPGPTRKHYQPYAPPRDFAAYRSRVKFSRSADAPAYQQGQNQLYNELNLGRREEYDVLDKRRGRDPEMGGKPRRKNPQEGLYNELQKDKMAEAYSEIGMKGERRRGKGHDGLYQGLSTATKDTYDALHMQALPPR

SEQ ID NO: 89 - protein, 969 aa, Synthetic construct
MALPVTALLLPLALLLHAARPEVQLVESGAEVKKPGASVKVSCKVSGYTLTELSMHWVRQAPGKGLEWMGGFDPEDGETMYAQKFQGRVTMTEDTSTDTAYMELSSLRSEDTAVYYCATSTAVAGTPDLFDYYYGMDVWGQGTTVTVSSGGGGSGGGGSGGGGSEIVMTQSPLSSPVTLGQPASISCRSSQSLVHSDGNTYLSWLQQRPGQPPRLLIYKISNRFSGVPDRFSGSGAGTDFTLKISRVEAEDVGVYYCTQATQFPYTFGQGTKVDIKDYKDDDDKQLSLPSILPNENEKVVQLNSSFSLRCFGESEVSWQYPMSEEESSDVEIRNEENNSGLFVTVLEVSSASAAHTGLYTCYYNHTQTEENELEGRHIYIYVPDPDVAFVPLGMTDYLVIVEDDDSAIIPCRTTDPETPVTLHNSEGVVPASYDSRQGFNGTFTVGPYICEATVKGKKFQTIPFNVYALKATSELDLEMEALKTVYKSGETIVVTCAVFNNEVVDLQWTYPGEVKGKGITMLEEIKVPSIKLVYTLTVPEATVKDSGDYECAARQATREVKEMKKVTISVHEKGFIEIKPTFSQLEAVNLHEVKHFVVEVRAYPPPRISWLKNNLTLIENLTEITTDVEKIQEIRYRSKLKLIRAKEEDSGHYTIVAQNEDAVKSYTFELLTQVPSSILDLVDDHHGSTGGQTVRCTAEGTPLPDIEWMICKDIKKCNNETSWTILANNVSNIITEIHSRDRSTVEGRVTFAKVEETIAVRCLAKNLLGAENRELKLVAPTLRSELTVAFWVLVVVGGVLACYSLLVTVAFIIFWVRSKRSRGGHSDYMNMTPRRPGPTRKHYQPYAPPRDFAAYRSRVKFSRSADAPAYQQGQNQLYNELNLGRREEYDVLDKRRGRDPEMGGKPRRKNPQEGLYNELQKDKMAEAYSEIGMKGERRRGKGHDGLYQGLSTATKDTYDALHMQALPPR

SEQ ID NO: 90 - protein, 964 aa, Synthetic construct
MALPVTALLLPLALLLHAARPEVQLVESGAEVKKPGASVKVSCKVSGYTLTELSMHWVRQAPGKGLEWMGGFDPEDGETMYAQKFQGRVTMTEDTSTDTAYMELSSLRSEDTAVYYCATSTAVAGTPDLFDYYYGMDVWGQGTTVTVSSGGGGSGGGGSGGGGSEIVMTQSPLSSPVTLGQPASISCRSSQSLVHSDGNTYLSWLQQRPGQPPRLLIYKISNRFSGVPDRFSGSGAGTDFTLKISRVEAEDVGVYYCTQATQFPYTFGQGTKVDIKDYKDDDDKLVVTPPGPELVLNVSSTFVLTCSGSAPVVWERMSQEPPQEMAKAQDGTFSSVLTLTNLTGLDTGEYFCTHNDSRGLETDERKRLYIFVPDPTVGFLPNDAEELFIFLTEITEITIPCRVTDPQLVVTLHEKKGDVALPVPYDHQRGFFGIFEDRSYICKTTIGDREVDSDAYYVYRLQVSSINVSVNAVQTVVRQGENITLMCIVIGNEVVNFEWTYPRKESGRLVEPVTDFLLDMPYHIRSILHIPSAELEDSGTYTCNVTESVNDHQDEKAINITVVESGYVRLLGEVGTLQFAELHRSRTLQVVFEAYPPPTVLWFKDNRTLGDSSAGEIALSTRNVSETRYVSELTLVRVKVAEAGHYTMRAFHEDAEVQLSFQLQINVPVRVLELSESHPDSGEQTVRCRGRGMPQPNIIWSACRDLKRCPRELPPTLLGNSSEEESQLETNVTYWEEEQEFEVVSTLRLQHVDRPLSVRCTLRNAVGQDTQEVIVVPHSLPFKVFWVLVVVGGVLACYSLLVTVAFIIFWVRSKRSRGGHSDYMNMTPRRPGPTRKHYQPYAPPRDFAAYRSRVKFSRSADAPAYQQGQNQLYNELNLGRREEYDVLDKRRGRDPEMGGKPRRKNPQEGLYNELQKDKMAEAYSEIGMKGERRRGKGHDGLYQGLSTATKDTYDALHMQALPPR

SEQ ID NO: 91 - protein, 608 aa, Synthetic construct
MALPVTALLLPLALLLHAARPEVQLVESGAEVKKPGASVKVSCKVSGYTLTELSMHWVRQAPGKGLEWMGGFDPEDGETMYAQKFQGRVTMTEDTSTDTAYMELSSLRSEDTAVYYCATSTAVAGTPDLFDYYYGMDVWGQGTTVTVSSGGGGSGGGGSGGGGSEIVMTQSPLSSPVTLGQPASISCRSSQSLVHSDGNTYLSWLQQRPGQPPRLLIYKISNRFSGVPDRFSGSGAGTDFTLKISRVEAEDVGVYYCTQATQFPYTFGQGTKVDIKDYKDDDDKQEEDLPRPSISAEPGTVIPLGSHVTFVCRGPVGVQTFRLERESRSTYNDTEDVSQASPSESEARFRIDSVSEGNAGPYRCIYYKPPKWSEQSDYLELLVKETSGGPDSPDTEPGSSAGPTQRPSDNSHNEHAPASQGLKAEHLYFWVLVVVGGVLACYSLLVTVAFIIFWVRSKRSRGGHSDYMNMTPRRPGPTRKHYQPYAPPRDFAAYRSRVKFSRSADAPAYQQGQNQLYNELNLGRREEYDVLDKRRGRDPEMGGKPRRKNPQEGLYNELQKDKMAEAYSEIGMKGERRRGKGHDGLYQGLSTATKDTYDALHMQALPPR

SEQ ID NO: 92 - protein, 512 aa, Synthetic construct
MALPVTALLLPLALLLHAARPEVQLVESGAEVKKPGASVKVSCKVSGYTLTELSMHWVRQAPGKGLEWMGGFDPEDGETMYAQKFQGRVTMTEDTSTDTAYMELSSLRSEDTAVYYCATSTAVAGTPDLFDYYYGMDVWGQGTTVTVSSGGGGSGGGGSGGGGSEIVMTQSPLSSPVTLGQPASISCRSSQSLVHSDGNTYLSWLQQRPGQPPRLLIYKISNRFSGVPDRFSGSGAGTDFTLKISRVEAEDVGVYYCTQATQFPYTFGQGTKVDIKDYKDDDDKLLVKETSGGPDSPDTEPGSSAGPTQRPSDNSHNEHAPASQGLKAEHLYFWVLVVVGGVLACYSLLVTVAFIIFWVRSKRSRGGHSDYMNMTPRRPGPTRKHYQPYAPPRDFAAYRSRVKFSRSADAPAYQQGQNQLYNELNLGRREEYDVLDKRRGRDPEMGGKPRRKNPQEGLYNELQKDKMAEAYSEIGMKGERRRGKGHDGLYQGLSTATKDTYDALHMQALPPR

SEQ ID NO: 93 - protein, 679 aa, Synthetic construct
MALPVTALLLPLALLLHAARPDIQMTQSPSSLSASVGDRVTITCRASQSISSYLNWYQQKPGKAPKLLIYAASSLQSGVPSRFSGSGSGTDFTLTISSLQPEDFATYYCQQSYSTPPTFGQGTKVEIKGGGGSGGGGSGGGGSEVQLVESGGGLVQPGGSLRLSCAASGFTFSDHYMDWVRQAPGKGLEWVGRTRNKANSYTTEYAASVKGRFTISRDDSKNSLYLQMNSLKTEDTAVYYCARGISPFYFDYWGQGTLVTVSSDYKDDDDKESKYGPPCPPCPAPPVAGPSVFLFPPKPKDTLMISRTPEVTCVVVDVSQEDPEVQFNWYVDGVEVHNAKTKPREEQFQSTYRVVSVLTVLHQDWLNGKEYKCKVSNKGLPSSIEKTISKAKGQPREPQVYTLPPSQEEMTKNQVSLTCLVKGFYPSDIAVEWESNGQPENNYKTTPPVLDSDGSFFLYSRLTVDKSRWQEGNVFSCSVMHEALHNHYTQKSLSLSLGKFWVLVVVGGVLACYSLLVTVAFIIFWVRSKRSRGGHSDYMNMTPRRPGPTRKHYQPYAPPRDFAAYRSRVKFSRSADAPAYQQGQNQLYNELNLGRREEYDVLDKRRGRDPEMGGKPRRKNPQEGLYNELQKDKMAEAYSEIGMKGERRRGKGHDGLYQGLSTATKDTYDALHMQALPPR

SEQ ID NO: 94 - protein, 12 aa, Synthetic construct
ASSSGYLFHSDY

SEQ ID NO: 95 - protein, 9 aa, Synthetic construct
QQYNSYPWT

SEQ ID NO: 96 - protein, 8 aa, Synthetic construct
GYTLTELS

SEQ ID NO: 97 - protein, 8 aa, Synthetic construct
FDPEDGET

SEQ ID NO: 98 - protein, 21 aa, Synthetic construct
ATSTAVAGTPDLFDYYYGMDV

SEQ ID NO: 99 - protein, 11 aa, Synthetic construct
QSLVHSDGNTY

SEQ ID NO: 100 - skipped

SEQ ID NO: 101 - protein, 9 aa, Synthetic construct
TQATQFPYT

SEQ ID NO: 102 - protein, 8 aa, Synthetic construct
FSDHYMDW

SEQ ID NO: 103 - protein, 22 aa, Synthetic construct
VGRTRNKANSYTTEYAASVKGR

SEQ ID NO: 104 - protein, 13 aa, Synthetic construct
CARGISPFYFDYW

SEQ ID NO: 105 - protein, 13 aa, Synthetic construct
CRASQSISSYLNW

SEQ ID NO: 106 - protein, 9 aa, Synthetic construct
YAASSLQSG

SEQ ID NO: 107 - protein, 11 aa, Synthetic construct
CQQSYSTPPTF

SEQ ID NO: 108 - protein, 1270 aa, Synthetic construct
MFVFLVLLPLVSSQCVNLTTRTQLPPAYTNSFTRGVYYPDKVFRSSVLHSTQDLFLPFFSNVTWFHVISGTNGTKRFDNPVLPFNDGVYFASIEKSNIIRGWIFGTTLDSKTQSLLIVNNATNVVIKVCEFQFCNDPFLDHKNNKSWMESEFRVYSSANNCTFEYVSQPFLMDLEGKQGNFKNLREFVFKNIDGYFKIYSKHTPIIVREPEDLPQGFSALEPLVDLPIGINITRFQTLLALHRSYLTPGDSSSGWTAGAAAYYVGYLQPRTFLLKYNENGTITDAVDCALDPLSETKCTLKSFTVEKGIYQTSNFRVQPTESIVRFPNITNLCPFDEVFNATRFASVYAWNRKRISNCVADYSVLYNLAPFFTFKCYGVSPTKLNDLCFTNVYADSFVIRGDEVRQIAPGQTGNIADYNYKLPDDFTGCVIAWNSNKLDSKVSGNYNYRYRLFRKSNLKPFERDISTEIYQAGNKPCNGVAGVNCYFPLQSYSFRPTYGVGHQPYRVVVLSFELLHAPATVCGPKKSTNLVKNKCVNFNFNGLKGTGVLTESNKKFLPFQQFGRDIADTTDAVRDPQTLEILDITPCSFGGVSVITPGTNTSNQVAVLYQGVNCTEVPVAIHADQLTPTWRVYSTGSNVFQTRAGCLIGAEYVNNSYECDIPIGAGICASYQTQTKSHRRARSVASQSIIAYTMSLGAENSVAYSNNSIAIPTNFTISVTTEILPVSMTKTSVDCTMYICGDSTECSNLLLQYGSFCTQLKRALTGIAVEQDKNTQEVFAQVKQIYKTPPIKYFGGFNFSQILPDPSKPSKRSFIEDLLFNKVTLADAGFIKQYGDCLGDIAARDLICAQKFKGLTVLPPLLTDEMIAQYTSALLAGTITSGWTFGAGAALQIPFAMQMAYRFNGIGVTQNVLYENQKLIANQFNSAIGKIQDSLSSTASALGKLQDVVNHNAQALNTLVKQLSSKFGAISSVLNDIFSRLDKVEAEVQIDRLITGRLQSLQTYVTQQLIRAAEIRASANLAATKMSECVLGQSKRVDFCGKGYHLMSFPQSAPHGVVFLHVTYVPAQEKNFTTAPAICHDGKAHFPREGVFVSNGTHWFVTQRNFYEPQIITTDNTFVSGNCDVVIGIVNNTVYDPLQPELDSFKEELDKYFKNHTSPDVDLGDISGINASVVNIQKEIDRLNEVAKNLNESLIDLQELGKYEQYIKWPWYIWLGFIAGLIAIVMVTIMLCCMTSCCSCLKGCCSCGSCCKFDEDDSEPVLKGVKLHYT

SEQ ID NO: 109 - protein, 42 aa, Synthetic construct
KRGRKKLLYIFKQPFMRPVQTTQEEDGCSCRFPEEEEGGCEL

SEQ ID NO: 110 - protein, 120 aa, Synthetic construct
WRRKRKEKQSETSPKEFLTIYEDVKDLKTRRNHEQEQTFPGGGSTIYSMIQSQSSAPTSQEPAYTLYSLIQPSRKSGSRKRNHSPSFNSTIYEVIGKSQPKAQNPARLSRKELENFDVYS

SEQ ID NO: 111 - DNA, 108 bp, synthetic construct
  source 1..108: mol_type = other DNA
agggaccagaggctgccccccgatgcccacaagccccctgggggaggcagtttccggacccccatccaagaggagcaggccgacgcccactccaccctggccaagatc

SEQ ID NO: 112 - protein, 556 aa, Synthetic construct [sequence omitted]

SEQ ID NO: 113 - protein, 557 aa, Synthetic construct
MPPPRLLFFLLFLTPMEVRPEEPLVVKVEEGDNAVLQCLKGTSDGPTQQLTWSRESPLKPFLKLSLGLPGLGIHMRPLAIWLFIFNVSQQMGGFYLCQPGPPSEKAWQPGWTVNVEGSGELFRWNVSDLGGLGCGLKNRSSEGPSSPSGKLMSPKLYVWAKDRPEIWEGEPPCLPPRDSLNQSLSQDLTMAPGSTLWLSCGVPPDSVSRGPLSWTHVHPKGPKSLLSLELKDDRPARDMWVMETGLLLPRATAQDAGKYYCHRGNLTMSFHLEITARPVLWHWLLRTGGWKVSAVTLAYLIFCLCSLVGILHLQRALVLRRKRKRMTDPTRRFFKVTPPPGSGPQNQYGNVLSLPTPTSGLGRAQRWAAGLGGTAPSYGNPSSDVQADGALGSRSPPGVGPEEEEGEGYEEPDSEEDSEFYENDSNLGQDQLSQDGSGYENPEDEPLGPEDEDSFSNAESYENEDEELTQPVARTMDFLSPHGSAWDPSREATSLAGSQSYEDMRGILYAAPQLRSIRGQPGPNHEEDADSYENMDNPDGPDPAWGGGGRMGTWSTR

SEQ ID NO: 114 - DNA, 105 bp, synthetic construct
  source 1..105: mol_type = other DNA
acaaaaaagaagtattcatccagtgtgcacgaccctaacggtgaatacatgttcatgagagcagtgaacacagccaaaaaatccagactcacagatgtgacccta

SEQ ID NO: 115 - protein, 20 aa, Synthetic construct
RPRRSPAQDGKVYINMPGRG

SEQ ID NO: 116 - protein, 21 aa, Synthetic construct
ESPYQELQGQRSDVYSDLNTQ

SEQ ID NO: 117 - protein, 5 aa, Synthetic construct
GGGGS